European Patent Specification EP 3 952 890 B1, published January 21, 2026. Title: METHODS AND COMPOSITIONS FOR PROGRAMMING T CELL DIFFERENTIATION AND ENHANCING T CELL PROLIFERATION. Applicant: THE TRUSTEES OF THE UNIVERSITY OF PENNSYLVANIA POWELL, Daniel SMOLE, Anze. Application PCT/US2020/027076. The sequence listing filed with the application follows.

SEQUENCE LISTING (40 sequences)

SEQ ID NO: 1 - DNA, 6 bp, Artificial Sequence
  Synthetic Construct
catatg

SEQ ID NO: 2 - DNA, 6 bp, Artificial Sequence
  Synthetic Construct
cccggg

SEQ ID NO: 3 - DNA, 264 bp, Artificial Sequence
  Synthetic Construct
ggtggctttaccaacagtaccggaatgcccccgggctggaagtcgagcttccattatataccctctaactagtacgccttctgtatgaaacagtttttcctccacgccttctgtatgaaacagtttttcctccacgccttctgtatgaaacagtttttcctccacgccttctgtatgaaacagtttttcctccacgccttctgtatgaaacagtttttcctccacgccttctgtatgaaacagtttttcctccaacagtaccgg

SEQ ID NO: 4 - DNA, 4908 bp, Artificial Sequence
  pASP73 (iFOX01-3A + Her2 CAR)
ttagccggaaacccagctgtgtgtggtggttttcacgctgtgagggaagctctggttgggcagcacgttatcgaagttgaagtccagggtatcgccgtccatcaggtcgttgcggatgatggattccatgtcgcagtccagtctctcgatgaacatgccgtccagatcagagggcagcttctcttggtgcagcaggcccattctgccgtagccattacagctggacacgctggagtagccgccgagggcagacatctgcataggatgaggcagtgggacctgcacaggggttttcacttgggtcagccggttcatgccgctggtatgaggcatggtggacacggtgtgaggcagaggtctgccattaacggcgcttgtctgctgggcatgtccagggtgtgtgtggctgctggggttcatcatcttgttgtggctggcctgagagccgtatgtgctcatcacgctattggggcccatcatcacgttctggcccagcactctactattaggctgggccacgccagggtccacaggtgtcatgatgtcgttgtgaggagggctgtcagaggtcagcagctctttcagcagtccaggggcacaattgtactggctcatgccgccgtaggaggacttgttgtcctgcagggtctgaatgggcatctgtggcagagggctcatgctgctctggccgtaggtgtacttctggtagttaggagatgggctgttcaggcttgtgttaggaggggcgaagctgtagcaaggggtctgctgcatcatggtgccggggctgctttgtgtagacacggtcaggctggtagggctgctcagcagattcaggttgtccagcaggttttccatgttctcggggttgctgatctcgctcaggcttggcagtgtgctggccattttggcggcgcttggaggatacaccatgctgtgcacgtcgccttctccgagatcatcctgctcggtcatgatggggctcagtctgccagagatggtgctggcattggcgctggttctgggtctgaaggtggaccagttgtcgaagtcgtcgttgctgtgagagccaggagaggcgggccacttagaaaactggctgccaggagaatcgccagcgccttcttgtccagactgcagagaggccttcttcttggcggctctgcttctgctcttggcgaacttggagttgttgtccatggcagcggcccttctacgaggagacttgccgctcttgccgccttcgggattcagcatccaccaagaggacttgccggtgccttcattctgcacccggatgaacttgctgtgcagggacagattgtgccggatgctgttcttccagccggcggagctattgctgtcgcccttgtccttgaagtagggcacgctcttgaccatccactcgtagatctggctcagggtcagtctcttctcggcgctgctctcaatggccttggtgatcaggtcggcgtagctcagattgccccaggcgtttcttctgctggagctgctctttctaggctgtccagcaagtggtccagcggcagctggaggaacaggaggatgctgagacagaggtccaggtggaggtggttgaggtggagcagggtgcagacatccggcctcaggtccctgaaaatcgccgcaaagtccacctgtagcagcagctgcggctgcggcggcaacagctgcagccacagatccaggagcctgagggaagtcctcgctctcttccagcaggctcaggttgctcatgaagtcggcggacactgcagcagcagaggcagaaggcagtccagcagcagcatcaggattagcggcggcagatccgctaggagcagggctagatgtggcgctgttgctctggctgaactcaggtctaggcagaggccaagcacaagatctaggccgaggcaggggctcgaaatcagggtcgatttccaccacctggggagcctcggccatggtggctttaccaacagtaccggaatgcccccgggctggaagtcgagcttccattatataccctctaactagtacgccttctgtatgaaacagtttttcctccacgccttctgtatgaaacagtttttcctccacgccttctgtatgaaacagtttttcctccacgccttctgtatgaaacagtttttcctccacgccttctgtatgaaacagtttttcctccacgccttctgtatgaaacagtttttcctccaacagtaccggatgcatcgtgaggctccggtgcccgtcagtgggcagagcgcacatcgcccacagtccccgagaagttggggggaggggtcggcaattgaaccggtgcctagagaaggtggcgcggggtaaactgggaaagtgatgtcgtgtactggctccgcctttttcccgagggtgggggagaaccgtatataagtgcagtagtcgccgtgaacgttctttttcgcaacgggtttgccgccagaacacaggtaagtgccgtgtgtggttcccgcgggcctggcctctttacgggttatggcccttgcgtgccttgaattacttccacctggctgcagtacgtgattcttgatcccgagcttcgggttggaagtgggtgggagagttcgaggccttgcgcttaaggagccccttcgcctcgtgcttgagttgaggcctggcctgggcgctggggccgccgcgtgcgaatctggtggcaccttcgcgcctgtctcgctgctttcgataagtctctagccatttaaaatttttgatgacctgctgcgacgctttttttctggcaagatagtcttgtaaatgcgggccaagatctgcacactggtatttcggtttttggggccgcgggcggcgacggggcccgtgcgtcccagcgcacatgttcggcgaggcggggcctgcgagcgcggccaccgagaatcggacgggggtagtctcaagctggccggcctgctctggtgcctggcctcgcgccgccgtgtatcgccccgccctgggcggcaaggctggcccggtcggcaccagttgcgtgagcggaaagatggccgcttcccggccctgctgcagggagctcaaaatggaggacgcggcgctcgggagagcgggcgggtgagtcacccacacaaaggaaaagggcctttccgtcctcagccgtcgcttcatgtgactccactgagtaccgggcgccgtccaggcacctcgattagttctcgtgcttttggagtacgtcgtctttaggttggggggaggggttttatgcgatggagtttccccacactgagtgggtggagactgaagttaggccagcttggcacttgatgtaattctccttggaatttgccctttttgagtttggatcttggttcattctcaagcctcagacagtggttcaaagtttttttcttccatttcaggtgtcgtgattctagagccaccatggccttaccagtgaccgccttgctcctgccgctggccttgctgctccacgccgccaggccggacattcaaatgacacagagtccctcatccctcagtgccagcgtgggcgatcgggtgactataacctgcagagcttctcaggacgtgaataccgctgtggcgtggtaccagcagaagccaggcaaagcgcctaagcttctcatttatagtgccagcttcctgtactcaggtgttccgtctcgcttttctggaagtagaagtgggaccgatttcacattgacgatcagcagcttgcagcccgaagatttcgccacctactactgtcagcagcactacactaccccaccgacatttggtcaaggcacaaaagtagagattaaacgcactggttccaccagcgggagcgggaaacccggctctggggaggggagcgaggtccagctggtggaatccgggggtggtcttgtgcagccaggaggatccttgaggttgtcctgcgccgcaagcggctttaacatcaaagatacatacatccattgggtccgacaggcccctggaaagggcctggagtgggtcgcccggatctacccaactaacgggtacactcgctacgctgatagcgtcaagggtcggtttactatttctgccgacacctcaaaaaacacagcctacctccagatgaactctctcagagctgaggatacagccgtgtactattgcagccggtggggaggcgacgggttctacgctatggatgtgtgggggcagggcacactggtcaccgtgagctcatccggaaccacgacgccagcgccgcgaccaccaacaccggcgcccaccatcgcgtcgcagcccctgtccctgcgcccagaggcgtgccggccagcggcggggggcgcagtgcacacgagggggctggacttcgcctgtgatatctacatctgggcgcccttggccgggacttgtggggtccttctcctgtcactggttatcaccctttactgcaaacggggcagaaagaaactcctgtatatattcaaacaaccatttatgagaccagtacaaactactcaagaggaagatggctgtagctgccgatttccagaagaagaagaaggaggatgtgaactgagagtgaagttcagcaggagcgcagacgcccccgcgtacaagcagggccagaaccagctctataacgagctcaatctaggacgaagagaggagtacgatgttttggacaagagacgtggccgggaccctgagatggggggaaagccgagaaggaagaaccctcaggaaggcctgtacaatgaactgcagaaagataagatggcggaggcctacagtgagattgggatgaaaggcgagcgccggaggggcaaggggcacgatggcctttaccagggtctcagtacagccaccaaggacacctacgacgcccttcacatgcaggccctgccccctcgctaa

SEQ ID NO: 5 - DNA, 180 bp, Artificial Sequence
  Synthetic NFAT promoter
ggaggaaaaactgtttcatacagaaggcgtggaggaaaaactgtttcatacagaaggcgtggaggaaaaactgtttcatacagaaggcgtggaggaaaaactgtttcatacagaaggcgtggaggaaaaactgtttcatacagaaggcgtggaggaaaaactgtttcatacagaaggcgt

SEQ ID NO: 6 - DNA, 32 bp, Artificial Sequence
  Minimal promoter
tagagggtatataatggaagctcgacttccag

SEQ ID NO: 7 - DNA, 1184 bp, Artificial Sequence
  EF1alpha promoter
cgtgaggctccggtgcccgtcagtgggcagagcgcacatcgcccacagtccccgagaagttggggggaggggtcggcaattgaaccggtgcctagagaaggtggcgcggggtaaactgggaaagtgatgtcgtgtactggctccgcctttttcccgagggtgggggagaaccgtatataagtgcagtagtcgccgtgaacgttctttttcgcaacgggtttgccgccagaacacaggtaagtgccgtgtgtggttcccgcgggcctggcctctttacgggttatggcccttgcgtgccttgaattacttccacctggctgcagtacgtgattcttgatcccgagcttcgggttggaagtgggtgggagagttcgaggccttgcgcttaaggagccccttcgcctcgtgcttgagttgaggcctggcctgggcgctggggccgccgcgtgcgaatctggtggcaccttcgcgcctgtctcgctgctttcgataagtctctagccatttaaaatttttgatgacctgctgcgacgctttttttctggcaagatagtcttgtaaatgcgggccaagatctgcacactggtatttcggtttttggggccgcgggcggcgacggggcccgtgcgtcccagcgcacatgttcggcgaggcggggcctgcgagcgcggccaccgagaatcggacgggggtagtctcaagctggccggcctgctctggtgcctggcctcgcgccgccgtgtatcgccccgccctgggcggcaaggctggcccggtcggcaccagttgcgtgagcggaaagatggccgcttcccggccctgctgcagggagctcaaaatggaggacgcggcgctcgggagagcgggcgggtgagtcacccacacaaaggaaaagggcctttccgtcctcagccgtcgcttcatgtgactccactgagtaccgggcgccgtccaggcacctcgattagttctcgtgcttttggagtacgtcgtctttaggttggggggaggggttttatgcgatggagtttccccacactgagtgggtggagactgaagttaggccagcttggcacttgatgtaattctccttggaatttgccctttttgagtttggatcttggttcattctcaagcctcagacagtggttcaaagtttttttcttccatttcaggtgtcgtga

SEQ ID NO: 8 - DNA, 29 bp, Artificial Sequence
  Spacer + Kozak sequence
ggcattccggtactgttggtaaagccacc

SEQ ID NO: 9 - DNA, 253 bp, Artificial Sequence
  Synthetic Construct
ggaggaaaaactgtttcatacagaaggcgtggaggaaaaactgtttcatacagaaggcgtggaggaaaaactgtttcatacagaaggcgtggaggaaaaactgtttcatacagaaggcgtggaggaaaaactgtttcatacagaaggcgtggaggaaaaactgtttcatacagaaggcgtactagttagagggtatataatggaagctcgacttccagcccgggggcattccggtactgttggtaaagccacc

SEQ ID NO: 10 - DNA, 2936 bp, Artificial Sequence
  pASP4.2
tcgagttaattaagctagcccggtactgttggaggaaaaactgtttcatacagaaggcgtggaggaaaaactgtttcatacagaaggcgtggaggaaaaactgtttcatacagaaggcgtggaggaaaaactgtttcatacagaaggcgtggaggaaaaactgtttcatacagaaggcgtggaggaaaaactgtttcatacagaaggcgtactagttagagggtatataatggaagctcgacttccagcccgggggcattccggtactgttggtaaagccaccatggtgagcaagggcgaggagctgttcaccggggtggtgcccatcctggtcgagctggacggcgacgtaaacggccacaagttcagcgtgtccggcgagggcgagggcgatgccacctacggcaagctgaccctgaagttcatctgcaccaccggcaagctgcccgtgccctggcccaccctcgtgaccaccctgacctacggcgtgcagtgcttcagccgctaccccgaccacatgaagcagcacgacttcttcaagtccgccatgcccgaaggctacgtccaggagcgcaccatcttcttcaaggacgacggcaactacaagacccgcgccgaggtgaagttcgagggcgacaccctggtgaaccgcatcgagctgaagggcatcgacttcaaggaggacggcaacatcctggggcacaagctggagtacaactacaacagccacaacgtctatatcatggccgacaagcagaagaacggcatcaaggtgaacttcaagatccgccacaacatcgaggacggcagcgtgcagctcgccgaccactaccagcagaacacccccatcggcgacggccccgtgctgctgcccgacaaccactacctgagcacccagtccgccctgagcaaagaccccaacgagaagcgcgatcacatggtcctgctggagttcgtgaccgccgccgggatcactctcggcatggacgagctgtacaagtaaatgcatcgtgaggctccggtgcccgtcagtgggcagagcgcacatcgcccacagtccccgagaagttggggggaggggtcggcaattgaaccggtgcctagagaaggtggcgcggggtaaactgggaaagtgatgtcgtgtactggctccgcctttttcccgagggtgggggagaaccgtatataagtgcagtagtcgccgtgaacgttctttttcgcaacgggtttgccgccagaacacaggtaagtgccgtgtgtggttcccgcgggcctggcctctttacgggttatggcccttgcgtgccttgaattacttccacctggctgcagtacgtgattcttgatcccgagcttcgggttggaagtgggtgggagagttcgaggccttgcgcttaaggagccccttcgcctcgtgcttgagttgaggcctggcctgggcgctggggccgccgcgtgcgaatctggtggcaccttcgcgcctgtctcgctgctttcgataagtctctagccatttaaaatttttgatgacctgctgcgacgctttttttctggcaagatagtcttgtaaatgcgggccaagatctgcacactggtatttcggtttttggggccgcgggcggcgacggggcccgtgcgtcccagcgcacatgttcggcgaggcggggcctgcgagcgcggccaccgagaatcggacgggggtagtctcaagctggccggcctgctctggtgcctggcctcgcgccgccgtgtatcgccccgccctgggcggcaaggctggcccggtcggcaccagttgcgtgagcggaaagatggccgcttcccggccctgctgcagggagctcaaaatggaggacgcggcgctcgggagagcgggcgggtgagtcacccacacaaaggaaaagggcctttccgtcctcagccgtcgcttcatgtgactccactgagtaccgggcgccgtccaggcacctcgattagttctcgtgcttttggagtacgtcgtctttaggttggggggaggggttttatgcgatggagtttccccacactgagtgggtggagactgaagttaggccagcttggcacttgatgtaattctccttggaatttgccctttttgagtttggatcttggttcattctcaagcctcagacagtggttcaaagtttttttcttccatttcaggtgtcgtgattctagagccaccatggtgagcaagggcgaggaggataacatggccatcatcaaggagttcatgcgcttcaaggtgcacatggagggctccgtgaacggccacgagttcgagatcgagggcgagggcgagggccgcccctacgagggcacccagaccgccaagctgaaggtgaccaagggtggccccctgcccttcgcctgggacatcctgtcccctcagttcatgtacggctccaaggcctacgtgaagcaccccgccgacatccccgactacttgaagctgtccttccccgagggcttcaagtgggagcgcgtgatgaacttcgaggacggcggcgtggtgaccgtgacccaggactcctccctgcaggacggcgagttcatctacaaggtgaagctgcgcggcaccaacttcccctccgacggccccgtaatgcagaagaagaccatgggctgggaggcctcctccgagcggatgtaccccgaggacggcgccctgaagggcgagatcaagcagaggctgaagctgaaggacggcggccactacgacgctgaggtcaagaccacctacaaggccaagaagcccgtgcagctgcccggcgcctacaacgtcaacatcaagttggacatcacctcccacaacgaggactacaccatcgtggaacagtacgaacgcgccgagggccgccactccaccggcggcatggacgagctgtacaagagggccaagaggcgtacgtaag

SEQ ID NO: 11 - DNA, 2936 bp, Artificial Sequence
  pASP5
tcgagttaattaagctagcttacttgtacagctcgtccatgccgagagtgatcccggcggcggtcacgaactccagcaggaccatgtgatcgcgcttctcgttggggtctttgctcagggcggactgggtgctcaggtagtggttgtcgggcagcagcacggggccgtcgccgatgggggtgttctgctggtagtggtcggcgagctgcacgctgccgtcctcgatgttgtggcggatcttgaagttcaccttgatgccgttcttctgcttgtcggccatgatatagacgttgtggctgttgtagttgtactccagcttgtgccccaggatgttgccgtcctccttgaagtcgatgcccttcagctcgatgcggttcaccagggtgtcgccctcgaacttcacctcggcgcgggtcttgtagttgccgtcgtccttgaagaagatggtgcgctcctggacgtagccttcgggcatggcggacttgaagaagtcgtgctgcttcatgtggtcggggtagcggctgaagcactgcacgccgtaggtcagggtggtcacgagggtgggccagggcacgggcagcttgccggtggtgcagatgaacttcagggtcagcttgccgtaggtggcatcgccctcgccctcgccggacacgctgaacttgtggccgtttacgtcgccgtccagctcgaccaggatgggcaccaccccggtgaacagctcctcgcccttgctcaccatggtggctttaccaacagtaccggaatgcccccgggctggaagtcgagcttccattatataccctctaactagtacgccttctgtatgaaacagtttttcctccacgccttctgtatgaaacagtttttcctccacgccttctgtatgaaacagtttttcctccacgccttctgtatgaaacagtttttcctccacgccttctgtatgaaacagtttttcctccacgccttctgtatgaaacagtttttcctccaacagtaccggatgcatcgtgaggctccggtgcccgtcagtgggcagagcgcacatcgcccacagtccccgagaagttggggggaggggtcggcaattgaaccggtgcctagagaaggtggcgcggggtaaactgggaaagtgatgtcgtgtactggctccgcctttttcccgagggtgggggagaaccgtatataagtgcagtagtcgccgtgaacgttctttttcgcaacgggtttgccgccagaacacaggtaagtgccgtgtgtggttcccgcgggcctggcctctttacgggttatggcccttgcgtgccttgaattacttccacctggctgcagtacgtgattcttgatcccgagcttcgggttggaagtgggtgggagagttcgaggccttgcgcttaaggagccccttcgcctcgtgcttgagttgaggcctggcctgggcgctggggccgccgcgtgcgaatctggtggcaccttcgcgcctgtctcgctgctttcgataagtctctagccatttaaaatttttgatgacctgctgcgacgctttttttctggcaagatagtcttgtaaatgcgggccaagatctgcacactggtatttcggtttttggggccgcgggcggcgacggggcccgtgcgtcccagcgcacatgttcggcgaggcggggcctgcgagcgcggccaccgagaatcggacgggggtagtctcaagctggccggcctgctctggtgcctggcctcgcgccgccgtgtatcgccccgccctgggcggcaaggctggcccggtcggcaccagttgcgtgagcggaaagatggccgcttcccggccctgctgcagggagctcaaaatggaggacgcggcgctcgggagagcgggcgggtgagtcacccacacaaaggaaaagggcctttccgtcctcagccgtcgcttcatgtgactccactgagtaccgggcgccgtccaggcacctcgattagttctcgtgcttttggagtacgtcgtctttaggttggggggaggggttttatgcgatggagtttccccacactgagtgggtggagactgaagttaggccagcttggcacttgatgtaattctccttggaatttgccctttttgagtttggatcttggttcattctcaagcctcagacagtggttcaaagtttttttcttccatttcaggtgtcgtgattctagagccaccatggtgagcaagggcgaggaggataacatggccatcatcaaggagttcatgcgcttcaaggtgcacatggagggctccgtgaacggccacgagttcgagatcgagggcgagggcgagggccgcccctacgagggcacccagaccgccaagctgaaggtgaccaagggtggccccctgcccttcgcctgggacatcctgtcccctcagttcatgtacggctccaaggcctacgtgaagcaccccgccgacatccccgactacttgaagctgtccttccccgagggcttcaagtgggagcgcgtgatgaacttcgaggacggcggcgtggtgaccgtgacccaggactcctccctgcaggacggcgagttcatctacaaggtgaagctgcgcggcaccaacttcccctccgacggccccgtaatgcagaagaagaccatgggctgggaggcctcctccgagcggatgtaccccgaggacggcgccctgaagggcgagatcaagcagaggctgaagctgaaggacggcggccactacgacgctgaggtcaagaccacctacaaggccaagaagcccgtgcagctgcccggcgcctacaacgtcaacatcaagttggacatcacctcccacaacgaggactacaccatcgtggaacagtacgaacgcgccgagggccgccactccaccggcggcatggacgagctgtacaagagggccaagaggcgtacgtaag

SEQ ID NO: 12 - DNA, 3158 bp, Artificial Sequence
  pASP7
tcgagtaccacatttgtagaggttttacttgctttaaaaaacctcccacacctccccctgaacctgaaacataaaatgaatgcaattgttgttgttaacttgtttattgcagcttataatggttacaaataaagcaatagcatcacaaatttcacaaataaagcatttttttcactgcattctagttgtggtttgtccaaactcatcaatgtatcttatcatgtctgttaattaagctagcttacttgtacagctcgtccatgccgagagtgatcccggcggcggtcacgaactccagcaggaccatgtgatcgcgcttctcgttggggtctttgctcagggcggactgggtgctcaggtagtggttgtcgggcagcagcacggggccgtcgccgatgggggtgttctgctggtagtggtcggcgagctgcacgctgccgtcctcgatgttgtggcggatcttgaagttcaccttgatgccgttcttctgcttgtcggccatgatatagacgttgtggctgttgtagttgtactccagcttgtgccccaggatgttgccgtcctccttgaagtcgatgcccttcagctcgatgcggttcaccagggtgtcgccctcgaacttcacctcggcgcgggtcttgtagttgccgtcgtccttgaagaagatggtgcgctcctggacgtagccttcgggcatggcggacttgaagaagtcgtgctgcttcatgtggtcggggtagcggctgaagcactgcacgccgtaggtcagggtggtcacgagggtgggccagggcacgggcagcttgccggtggtgcagatgaacttcagggtcagcttgccgtaggtggcatcgccctcgccctcgccggacacgctgaacttgtggccgtttacgtcgccgtccagctcgaccaggatgggcaccaccccggtgaacagctcctcgcccttgctcaccatggtggctttaccaacagtaccggaatgcccccgggctggaagtcgagcttccattatataccctctaactagtacgccttctgtatgaaacagtttttcctccacgccttctgtatgaaacagtttttcctccacgccttctgtatgaaacagtttttcctccacgccttctgtatgaaacagtttttcctccacgccttctgtatgaaacagtttttcctccacgccttctgtatgaaacagtttttcctccaacagtaccggatgcatcgtgaggctccggtgcccgtcagtgggcagagcgcacatcgcccacagtccccgagaagttggggggaggggtcggcaattgaaccggtgcctagagaaggtggcgcggggtaaactgggaaagtgatgtcgtgtactggctccgcctttttcccgagggtgggggagaaccgtatataagtgcagtagtcgccgtgaacgttctttttcgcaacgggtttgccgccagaacacaggtaagtgccgtgtgtggttcccgcgggcctggcctctttacgggttatggcccttgcgtgccttgaattacttccacctggctgcagtacgtgattcttgatcccgagcttcgggttggaagtgggtgggagagttcgaggccttgcgcttaaggagccccttcgcctcgtgcttgagttgaggcctggcctgggcgctggggccgccgcgtgcgaatctggtggcaccttcgcgcctgtctcgctgctttcgataagtctctagccatttaaaatttttgatgacctgctgcgacgctttttttctggcaagatagtcttgtaaatgcgggccaagatctgcacactggtatttcggtttttggggccgcgggcggcgacggggcccgtgcgtcccagcgcacatgttcggcgaggcggggcctgcgagcgcggccaccgagaatcggacgggggtagtctcaagctggccggcctgctctggtgcctggcctcgcgccgccgtgtatcgccccgccctgggcggcaaggctggcccggtcggcaccagttgcgtgagcggaaagatggccgcttcccggccctgctgcagggagctcaaaatggaggacgcggcgctcgggagagcgggcgggtgagtcacccacacaaaggaaaagggcctttccgtcctcagccgtcgcttcatgtgactccactgagtaccgggcgccgtccaggcacctcgattagttctcgtgcttttggagtacgtcgtctttaggttggggggaggggttttatgcgatggagtttccccacactgagtgggtggagactgaagttaggccagcttggcacttgatgtaattctccttggaatttgccctttttgagtttggatcttggttcattctcaagcctcagacagtggttcaaagtttttttcttccatttcaggtgtcgtgattctagagccaccatggtgagcaagggcgaggaggataacatggccatcatcaaggagttcatgcgcttcaaggtgcacatggagggctccgtgaacggccacgagttcgagatcgagggcgagggcgagggccgcccctacgagggcacccagaccgccaagctgaaggtgaccaagggtggccccctgcccttcgcctgggacatcctgtcccctcagttcatgtacggctccaaggcctacgtgaagcaccccgccgacatccccgactacttgaagctgtccttccccgagggcttcaagtgggagcgcgtgatgaacttcgaggacggcggcgtggtgaccgtgacccaggactcctccctgcaggacggcgagttcatctacaaggtgaagctgcgcggcaccaacttcccctccgacggccccgtaatgcagaagaagaccatgggctgggaggcctcctccgagcggatgtaccccgaggacggcgccctgaagggcgagatcaagcagaggctgaagctgaaggacggcggccactacgacgctgaggtcaagaccacctacaaggccaagaagcccgtgcagctgcccggcgcctacaacgtcaacatcaagttggacatcacctcccacaacgaggactacaccatcgtggaacagtacgaacgcgccgagggccgccactccaccggcggcatggacgagctgtacaagagggccaagaggcgtacgtaag

SEQ ID NO: 13 - DNA, 3413 bp, Artificial Sequence
  pASP8
tcgagttaattaagctagcaaggctttctgtttcctgcattcttacttcttactacgtgatacatctagtcaccagggaagaagcgaatgacacacttccaaaaaccaattcgtagctttctaaataaaaccctttctagctggagagagatccatgagcatagagatcttaaaattcatgttcagcaataaatcctggggccccagacagtgtcaggtgcatagggggtgttcagtaaatatcagttaaatgttgcataaatccgataaacgggattcctggaaaatactacactctccttctccaaattatcttcatctcaaagacaggaacctctaacttttaattctttacttagattatgctgtctcctaaactgtttatgttttctgaaatttaaggcaggatgtctcagagtctgggaaaatcccactttcctcctgctacaccttacagttgtgagaaagcacatttcagacaacagggaaaacccatacttcaccacaacaacacactatacattgtctggtccactggagcataaattaaagagaaacaatgtagtcaagcaagtaggcggcaagaggaagggggcggagacatcatcagggagtataaactctgagatgcctcagagcctcacagactcaacaagagctccagcaaagactttcactgtagcttgacttgacctgagattaactagggaatcttgagaataaagcccgggggcattccggtactgttggtaaagccaccatggtgagcaagggcgaggagctgttcaccggggtggtgcccatcctggtcgagctggacggcgacgtaaacggccacaagttcagcgtgtccggcgagggcgagggcgatgccacctacggcaagctgaccctgaagttcatctgcaccaccggcaagctgcccgtgccctggcccaccctcgtgaccaccctgacctacggcgtgcagtgcttcagccgctaccccgaccacatgaagcagcacgacttcttcaagtccgccatgcccgaaggctacgtccaggagcgcaccatcttcttcaaggacgacggcaactacaagacccgcgccgaggtgaagttcgagggcgacaccctggtgaaccgcatcgagctgaagggcatcgacttcaaggaggacggcaacatcctggggcacaagctggagtacaactacaacagccacaacgtctatatcatggccgacaagcagaagaacggcatcaaggtgaacttcaagatccgccacaacatcgaggacggcagcgtgcagctcgccgaccactaccagcagaacacccccatcggcgacggccccgtgctgctgcccgacaaccactacctgagcacccagtccgccctgagcaaagaccccaacgagaagcgcgatcacatggtcctgctggagttcgtgaccgccgccgggatcactctcggcatggacgagctgtacaagtaaatgcatcgtgaggctccggtgcccgtcagtgggcagagcgcacatcgcccacagtccccgagaagttggggggaggggtcggcaattgaaccggtgcctagagaaggtggcgcggggtaaactgggaaagtgatgtcgtgtactggctccgcctttttcccgagggtgggggagaaccgtatataagtgcagtagtcgccgtgaacgttctttttcgcaacgggtttgccgccagaacacaggtaagtgccgtgtgtggttcccgcgggcctggcctctttacgggttatggcccttgcgtgccttgaattacttccacctggctgcagtacgtgattcttgatcccgagcttcgggttggaagtgggtgggagagttcgaggccttgcgcttaaggagccccttcgcctcgtgcttgagttgaggcctggcctgggcgctggggccgccgcgtgcgaatctggtggcaccttcgcgcctgtctcgctgctttcgataagtctctagccatttaaaatttttgatgacctgctgcgacgctttttttctggcaagatagtcttgtaaatgcgggccaagatctgcacactggtatttcggtttttggggccgcgggcggcgacggggcccgtgcgtcccagcgcacatgttcggcgaggcggggcctgcgagcgcggccaccgagaatcggacgggggtagtctcaagctggccggcctgctctggtgcctggcctcgcgccgccgtgtatcgccccgccctgggcggcaaggctggcccggtcggcaccagttgcgtgagcggaaagatggccgcttcccggccctgctgcagggagctcaaaatggaggacgcggcgctcgggagagcgggcgggtgagtcacccacacaaaggaaaagggcctttccgtcctcagccgtcgcttcatgtgactccactgagtaccgggcgccgtccaggcacctcgattagttctcgtgcttttggagtacgtcgtctttaggttggggggaggggttttatgcgatggagtttccccacactgagtgggtggagactgaagttaggccagcttggcacttgatgtaattctccttggaatttgccctttttgagtttggatcttggttcattctcaagcctcagacagtggttcaaagtttttttcttccatttcaggtgtcgtgattctagagccaccatggtgagcaagggcgaggaggataacatggccatcatcaaggagttcatgcgcttcaaggtgcacatggagggctccgtgaacggccacgagttcgagatcgagggcgagggcgagggccgcccctacgagggcacccagaccgccaagctgaaggtgaccaagggtggccccctgcccttcgcctgggacatcctgtcccctcagttcatgtacggctccaaggcctacgtgaagcaccccgccgacatccccgactacttgaagctgtccttccccgagggcttcaagtgggagcgcgtgatgaacttcgaggacggcggcgtggtgaccgtgacccaggactcctccctgcaggacggcgagttcatctacaaggtgaagctgcgcggcaccaacttcccctccgacggccccgtaatgcagaagaagaccatgggctgggaggcctcctccgagcggatgtaccccgaggacggcgccctgaagggcgagatcaagcagaggctgaagctgaaggacggcggccactacgacgctgaggtcaagaccacctacaaggccaagaagcccgtgcagctgcccggcgcctacaacgtcaacatcaagttggacatcacctcccacaacgaggactacaccatcgtggaacagtacgaacgcgccgagggccgccactccaccggcggcatggacgagctgtacaagagggccaagaggcgtacgtaag

SEQ ID NO: 14 - DNA, 3031 bp, Artificial Sequence
  pASP9
tcgagttaattaagctagcaatgctttgtcctggagagctatcttaagggacaaaatcgttttcccagcgtcatctgtgacacatcctgacagtagagagctgcttccaagaagcaatttgaagtgccattatcaggcagggacgggggctctaggggatttcggggtcagcagatatgaaatgaatgatttcatagggctgtcacagagctgtggtgggaatttcccatgagaccccgcccctggctgagtcaccgcactcctgtgtttgacctgaagtcctctcgtgctgcagaagcctgaagaccaaggagtggaaagttctccggcagccctgagatctcccgggggcattccggtactgttggtaaagccaccatggtgagcaagggcgaggagctgttcaccggggtggtgcccatcctggtcgagctggacggcgacgtaaacggccacaagttcagcgtgtccggcgagggcgagggcgatgccacctacggcaagctgaccctgaagttcatctgcaccaccggcaagctgcccgtgccctggcccaccctcgtgaccaccctgacctacggcgtgcagtgcttcagccgctaccccgaccacatgaagcagcacgacttcttcaagtccgccatgcccgaaggctacgtccaggagcgcaccatcttcttcaaggacgacggcaactacaagacccgcgccgaggtgaagttcgagggcgacaccctggtgaaccgcatcgagctgaagggcatcgacttcaaggaggacggcaacatcctggggcacaagctggagtacaactacaacagccacaacgtctatatcatggccgacaagcagaagaacggcatcaaggtgaacttcaagatccgccacaacatcgaggacggcagcgtgcagctcgccgaccactaccagcagaacacccccatcggcgacggccccgtgctgctgcccgacaaccactacctgagcacccagtccgccctgagcaaagaccccaacgagaagcgcgatcacatggtcctgctggagttcgtgaccgccgccgggatcactctcggcatggacgagctgtacaagtaaatgcatcgtgaggctccggtgcccgtcagtgggcagagcgcacatcgcccacagtccccgagaagttggggggaggggtcggcaattgaaccggtgcctagagaaggtggcgcggggtaaactgggaaagtgatgtcgtgtactggctccgcctttttcccgagggtgggggagaaccgtatataagtgcagtagtcgccgtgaacgttctttttcgcaacgggtttgccgccagaacacaggtaagtgccgtgtgtggttcccgcgggcctggcctctttacgggttatggcccttgcgtgccttgaattacttccacctggctgcagtacgtgattcttgatcccgagcttcgggttggaagtgggtgggagagttcgaggccttgcgcttaaggagccccttcgcctcgtgcttgagttgaggcctggcctgggcgctggggccgccgcgtgcgaatctggtggcaccttcgcgcctgtctcgctgctttcgataagtctctagccatttaaaatttttgatgacctgctgcgacgctttttttctggcaagatagtcttgtaaatgcgggccaagatctgcacactggtatttcggtttttggggccgcgggcggcgacggggcccgtgcgtcccagcgcacatgttcggcgaggcggggcctgcgagcgcggccaccgagaatcggacgggggtagtctcaagctggccggcctgctctggtgcctggcctcgcgccgccgtgtatcgccccgccctgggcggcaaggctggcccggtcggcaccagttgcgtgagcggaaagatggccgcttcccggccctgctgcagggagctcaaaatggaggacgcggcgctcgggagagcgggcgggtgagtcacccacacaaaggaaaagggcctttccgtcctcagccgtcgcttcatgtgactccactgagtaccgggcgccgtccaggcacctcgattagttctcgtgcttttggagtacgtcgtctttaggttggggggaggggttttatgcgatggagtttccccacactgagtgggtggagactgaagttaggccagcttggcacttgatgtaattctccttggaatttgccctttttgagtttggatcttggttcattctcaagcctcagacagtggttcaaagtttttttcttccatttcaggtgtcgtgattctagagccaccatggtgagcaagggcgaggaggataacatggccatcatcaaggagttcatgcgcttcaaggtgcacatggagggctccgtgaacggccacgagttcgagatcgagggcgagggcgagggccgcccctacgagggcacccagaccgccaagctgaaggtgaccaagggtggccccctgcccttcgcctgggacatcctgtcccctcagttcatgtacggctccaaggcctacgtgaagcaccccgccgacatccccgactacttgaagctgtccttccccgagggcttcaagtgggagcgcgtgatgaacttcgaggacggcggcgtggtgaccgtgacccaggactcctccctgcaggacggcgagttcatctacaaggtgaagctgcgcggcaccaacttcccctccgacggccccgtaatgcagaagaagaccatgggctgggaggcctcctccgagcggatgtaccccgaggacggcgccctgaagggcgagatcaagcagaggctgaagctgaaggacggcggccactacgacgctgaggtcaagaccacctacaaggccaagaagcccgtgcagctgcccggcgcctacaacgtcaacatcaagttggacatcacctcccacaacgaggactacaccatcgtggaacagtacgaacgcgccgagggccgccactccaccggcggcatggacgagctgtacaagagggccaagaggcgtacgtaag

SEQ ID NO: 15 - DNA, 3815 bp, Artificial Sequence
  pASP18
tcgagttaattaagctagcccggtactgttggaggaaaaactgtttcatacagaaggcgtggaggaaaaactgtttcatacagaaggcgtggaggaaaaactgtttcatacagaaggcgtggaggaaaaactgtttcatacagaaggcgtggaggaaaaactgtttcatacagaaggcgtggaggaaaaactgtttcatacagaaggcgtactagttagagggtatataatggaagctcgacttccagcccgggggcattccggtactgttggtaaagccaccatgtgccaccagcagctggtcatcagctggttcagcctggtgttcctggccagccctctggtggccatctgggagctgaagaaagacgtgtacgtggtggaactggactggtatcccgacgcccctggcgagatggtggtgctgacctgcgacacccctgaagaggacggcatcacctggaccctggaccagtctagcgaggtgctgggcagcggcaagaccctgaccatccaggtcaaagagttcggcgacgccggccagtacacctgtcacaagggcggagaggtgctgagccacagcctgctgctgctccacaagaaagaggatggcatttggagcaccgacatcctgaaggaccagaaagagcccaagaacaagaccttcctgagatgcgaggccaagaactacagcggccggttcacctgttggtggctgaccaccatcagcaccgacctgaccttcagcgtgaagtccagcagaggcagcagcgaccctcagggcgtgacatgtggcgccgctacactgtctgccgagagagtgcggggcgacaacaaagagtacgagtacagcgtcgagtgccaggaagatagcgcctgccctgccgccgaggaaagcctgcctatcgaagtgatggtggacgccgtgcacaagctgaagtacgagaactacacctccagctttttcatccgggacatcatcaagcccgaccctcccaagaacctgcagctgaagcctctgaagaacagcagacaggtggaagtgtcctgggagtaccccgacacctggtccacccctcacagctacttcagcctgacattctgtgtgcaagtccagggcaagtccaagcgcgagaaaaaggaccgggtgttcaccgacaagaccagcgccaccgtgatctgccggaagaacgcctctatcagcgtgcgggcccaggaccggtactacagcagctcttggagcgagtgggccagcgtgccatgttctggtggcggaggcggcggaagcagaaatctgccagtggccacccctgaccccggcatgtttccttgtctgcaccacagccagaacctgctgcgggccgtgtccaacatgctgcagaaggcccggcagaccctggaattctacccctgcaccagcgaggaaatcgaccacgaggacatcaccaaggataagaccagcaccgtggaagcctgtctgcccctggaactgaccaagaacgagagctgcctgaacagccgggaaaccagcttcatcaccaacggcagctgtctggccagcagaaagacctccttcatgatggccctgtgcctgagcagcatctacgaggacctgaagatgtaccaggtcgagttcaagaccatgaacgccaagctgctgatggaccccaagcggcagatctttctggaccagaatatgctggccgtgatcgacgagctgatgcaggccctgaacttcaacagcgagacagtgccccagaagtcctccctggaagaacccgacttctacaagaccaagatcaagctgtgcatcctgctgcacgccttccggatcagagccgtgaccatcgacagagtgatgagctacctgaacgcctcctaaatgcatcgtgaggctccggtgcccgtcagtgggcagagcgcacatcgcccacagtccccgagaagttggggggaggggtcggcaattgaaccggtgcctagagaaggtggcgcggggtaaactgggaaagtgatgtcgtgtactggctccgcctttttcccgagggtgggggagaaccgtatataagtgcagtagtcgccgtgaacgttctttttcgcaacgggtttgccgccagaacacaggtaagtgccgtgtgtggttcccgcgggcctggcctctttacgggttatggcccttgcgtgccttgaattacttccacctggctgcagtacgtgattcttgatcccgagcttcgggttggaagtgggtgggagagttcgaggccttgcgcttaaggagccccttcgcctcgtgcttgagttgaggcctggcctgggcgctggggccgccgcgtgcgaatctggtggcaccttcgcgcctgtctcgctgctttcgataagtctctagccatttaaaatttttgatgacctgctgcgacgctttttttctggcaagatagtcttgtaaatgcgggccaagatctgcacactggtatttcggtttttggggccgcgggcggcgacggggcccgtgcgtcccagcgcacatgttcggcgaggcggggcctgcgagcgcggccaccgagaatcggacgggggtagtctcaagctggccggcctgctctggtgcctggcctcgcgccgccgtgtatcgccccgccctgggcggcaaggctggcccggtcggcaccagttgcgtgagcggaaagatggccgcttcccggccctgctgcagggagctcaaaatggaggacgcggcgctcgggagagcgggcgggtgagtcacccacacaaaggaaaagggcctttccgtcctcagccgtcgcttcatgtgactccactgagtaccgggcgccgtccaggcacctcgattagttctcgtgcttttggagtacgtcgtctttaggttggggggaggggttttatgcgatggagtttccccacactgagtgggtggagactgaagttaggccagcttggcacttgatgtaattctccttggaatttgccctttttgagtttggatcttggttcattctcaagcctcagacagtggttcaaagtttttttcttccatttcaggtgtcgtgattctagagccaccatggtgagcaagggcgaggaggataacatggccatcatcaaggagttcatgcgcttcaaggtgcacatggagggctccgtgaacggccacgagttcgagatcgagggcgagggcgagggccgcccctacgagggcacccagaccgccaagctgaaggtgaccaagggtggccccctgcccttcgcctgggacatcctgtcccctcagttcatgtacggctccaaggcctacgtgaagcaccccgccgacatccccgactacttgaagctgtccttccccgagggcttcaagtgggagcgcgtgatgaacttcgaggacggcggcgtggtgaccgtgacccaggactcctccctgcaggacggcgagttcatctacaaggtgaagctgcgcggcaccaacttcccctccgacggccccgtaatgcagaagaagaccatgggctgggaggcctcctccgagcggatgtaccccgaggacggcgccctgaagggcgagatcaagcagaggctgaagctgaaggacggcggccactacgacgctgaggtcaagaccacctacaaggccaagaagcccgtgcagctgcccggcgcctacaacgtcaacatcaagttggacatcacctcccacaacgaggactacaccatcgtggaacagtacgaacgcgccgagggccgccactccaccggcggcatggacgagctgtacaagagggccaagaggcgtacgtaag

SEQ ID NO: 16 - DNA, 3680 bp, Artificial Sequence
  pASP26
tcgagttaattaagctagcccggtactgttggaggaaaaactgtttcatacagaaggcgtggaggaaaaactgtttcatacagaaggcgtggaggaaaaactgtttcatacagaaggcgtggaggaaaaactgtttcatacagaaggcgtggaggaaaaactgtttcatacagaaggcgtggaggaaaaactgtttcatacagaaggcgtactagttagagggtatataatggaagctcgacttccagcccgggggcattccggtactgttggtaaagccaccatggtgagcaagggcgaggagctgttcaccggggtggtgcccatcctggtcgagctggacggcgacgtaaacggccacaagttcagcgtgtccggcgagggcgagggcgatgccacctacggcaagctgaccctgaagttcatctgcaccaccggcaagctgcccgtgccctggcccaccctcgtgaccaccctgacctacggcgtgcagtgcttcagccgctaccccgaccacatgaagcagcacgacttcttcaagtccgccatgcccgaaggctacgtccaggagcgcaccatcttcttcaaggacgacggcaactacaagacccgcgccgaggtgaagttcgagggcgacaccctggtgaaccgcatcgagctgaagggcatcgacttcaaggaggacggcaacatcctggggcacaagctggagtacaactacaacagccacaacgtctatatcatggccgacaagcagaagaacggcatcaaggtgaacttcaagatccgccacaacatcgaggacggcagcgtgcagctcgccgaccactaccagcagaacacccccatcggcgacggccccgtgctgctgcccgacaaccactacctgagcacccagtccgccctgagcaaagaccccaacgagaagcgcgatcacatggtcctgctggagttcgtgaccgccgccgggatcactctcggcatggacgagctgtacaagtaaatgcatcgtgaggctccggtgcccgtcagtgggcagagcgcacatcgcccacagtccccgagaagttggggggaggggtcggcaattgaaccggtgcctagagaaggtggcgcggggtaaactgggaaagtgatgtcgtgtactggctccgcctttttcccgagggtgggggagaaccgtatataagtgcagtagtcgccgtgaacgttctttttcgcaacgggtttgccgccagaacacaggtaagtgccgtgtgtggttcccgcgggcctggcctctttacgggttatggcccttgcgtgccttgaattacttccacctggctgcagtacgtgattcttgatcccgagcttcgggttggaagtgggtgggagagttcgaggccttgcgcttaaggagccccttcgcctcgtgcttgagttgaggcctggcctgggcgctggggccgccgcgtgcgaatctggtggcaccttcgcgcctgtctcgctgctttcgataagtctctagccatttaaaatttttgatgacctgctgcgacgctttttttctggcaagatagtcttgtaaatgcgggccaagatctgcacactggtatttcggtttttggggccgcgggcggcgacggggcccgtgcgtcccagcgcacatgttcggcgaggcggggcctgcgagcgcggccaccgagaatcggacgggggtagtctcaagctggccggcctgctctggtgcctggcctcgcgccgccgtgtatcgccccgccctgggcggcaaggctggcccggtcggcaccagttgcgtgagcggaaagatggccgcttcccggccctgctgcagggagctcaaaatggaggacgcggcgctcgggagagcgggcgggtgagtcacccacacaaaggaaaagggcctttccgtcctcagccgtcgcttcatgtgactccactgagtaccgggcgccgtccaggcacctcgattagttctcgtgcttttggagtacgtcgtctttaggttggggggaggggttttatgcgatggagtttccccacactgagtgggtggagactgaagttaggccagcttggcacttgatgtaattctccttggaatttgccctttttgagtttggatcttggttcattctcaagcctcagacagtggttcaaagtttttttcttccatttcaggtgtcgtgattctagagccaccatggccttaccagtgaccgccttgctcctgccgctggccttgctgctccacgccgccaggccggacattcaaatgacacagagtccctcatccctcagtgccagcgtgggcgatcgggtgactataacctgcagagcttctcaggacgtgaataccgctgtggcgtggtaccagcagaagccaggcaaagcgcctaagcttctcatttatagtgccagcttcctgtactcaggtgttccgtctcgcttttctggaagtagaagtgggaccgatttcacattgacgatcagcagcttgcagcccgaagatttcgccacctactactgtcagcagcactacactaccccaccgacatttggtcaaggcacaaaagtagagattaaacgcactggttccaccagcgggagcgggaaacccggctctggggaggggagcgaggtccagctggtggaatccgggggtggtcttgtgcagccaggaggatccttgaggttgtcctgcgccgcaagcggctttaacatcaaagatacatacatccattgggtccgacaggcccctggaaagggcctggagtgggtcgcccggatctacccaactaacgggtacactcgctacgctgatagcgtcaagggtcggtttactatttctgccgacacctcaaaaaacacagcctacctccagatgaactctctcagagctgaggatacagccgtgtactattgcagccggtggggaggcgacgggttctacgctatggatgtgtgggggcagggcacactggtcaccgtgagctcatccggaaccacgacgccagcgccgcgaccaccaacaccggcgcccaccatcgcgtcgcagcccctgtccctgcgcccagaggcgtgccggccagcggcggggggcgcagtgcacacgagggggctggacttcgcctgtgatatctacatctgggcgcccttggccgggacttgtggggtccttctcctgtcactggttatcaccctttactgcaaacggggcagaaagaaactcctgtatatattcaaacaaccatttatgagaccagtacaaactactcaagaggaagatggctgtagctgccgatttccagaagaagaagaaggaggatgtgaactgagagtgaagttcagcaggagcgcagacgcccccgcgtacaagcagggccagaaccagctctataacgagctcaatctaggacgaagagaggagtacgatgttttggacaagagacgtggccgggaccctgagatggggggaaagccgagaaggaagaaccctcaggaaggcctgtacaatgaactgcagaaagataagatggcggaggcctacagtgagattgggatgaaaggcgagcgccggaggggcaaggggcacgatggcctttaccagggtctcagtacagccaccaaggacacctacgacgcccttcacatgcaggccctgccccctcgctaag

SEQ ID NO: 17 - DNA, 3689 bp, Artificial Sequence
  pASP28
tcgagttaattaagctagcttacttgtacagctcgtccatgccgagagtgatcccggcggcggtcacgaactccagcaggaccatgtgatcgcgcttctcgttggggtctttgctcagggcggactgggtgctcaggtagtggttgtcgggcagcagcacggggccgtcgccgatgggggtgttctgctggtagtggtcggcgagctgcacgctgccgtcctcgatgttgtggcggatcttgaagttcaccttgatgccgttcttctgcttgtcggccatgatatagacgttgtggctgttgtagttgtactccagcttgtgccccaggatgttgccgtcctccttgaagtcgatgcccttcagctcgatgcggttcaccagggtgtcgccctcgaacttcacctcggcgcgggtcttgtagttgccgtcgtccttgaagaagatggtgcgctcctggacgtagccttcgggcatggcggacttgaagaagtcgtgctgcttcatgtggtcggggtagcggctgaagcactgcacgccgtaggtcagggtggtcacgagggtgggccagggcacgggcagcttgccggtggtgcagatgaacttcagggtcagcttgccgtaggtggcatcgccctcgccctcgccggacacgctgaacttgtggccgtttacgtcgccgtccagctcgaccaggatgggcaccaccccggtgaacagctcctcgcccttgctcaccatggtggctttaccaacagtaccggaatgcccccgggctggaagtcgagcttccattatataccctctaactagtacgccttctgtatgaaacagtttttcctccacgccttctgtatgaaacagtttttcctccacgccttctgtatgaaacagtttttcctccacgccttctgtatgaaacagtttttcctccacgccttctgtatgaaacagtttttcctccacgccttctgtatgaaacagtttttcctccaacagtaccggatgcatcgtgaggctccggtgcccgtcagtgggcagagcgcacatcgcccacagtccccgagaagttggggggaggggtcggcaattgaaccggtgcctagagaaggtggcgcggggtaaactgggaaagtgatgtcgtgtactggctccgcctttttcccgagggtgggggagaaccgtatataagtgcagtagtcgccgtgaacgttctttttcgcaacgggtttgccgccagaacacaggtaagtgccgtgtgtggttcccgcgggcctggcctctttacgggttatggcccttgcgtgccttgaattacttccacctggctgcagtacgtgattcttgatcccgagcttcgggttggaagtgggtgggagagttcgaggccttgcgcttaaggagccccttcgcctcgtgcttgagttgaggcctggcctgggcgctggggccgccgcgtgcgaatctggtggcaccttcgcgcctgtctcgctgctttcgataagtctctagccatttaaaatttttgatgacctgctgcgacgctttttttctggcaagatagtcttgtaaatgcgggccaagatctgcacactggtatttcggtttttggggccgcgggcggcgacggggcccgtgcgtcccagcgcacatgttcggcgaggcggggcctgcgagcgcggccaccgagaatcggacgggggtagtctcaagctggccggcctgctctggtgcctggcctcgcgccgccgtgtatcgccccgccctgggcggcaaggctggcccggtcggcaccagttgcgtgagcggaaagatggccgcttcccggccctgctgcagggagctcaaaatggaggacgcggcgctcgggagagcgggcgggtgagtcacccacacaaaggaaaagggcctttccgtcctcagccgtcgcttcatgtgactccactgagtaccgggcgccgtccaggcacctcgattagttctcgtgcttttggagtacgtcgtctttaggttggggggaggggttttatgcgatggagtttccccacactgagtgggtggagactgaagttaggccagcttggcacttgatgtaattctccttggaatttgccctttttgagtttggatcttggttcattctcaagcctcagacagtggttcaaagtttttttcttccatttcaggtgtcgtgattctagaatggccttaccagtgaccgccttgctcctgccgctggccttgctgctccacgccgccaggccgggatccgacatcgttctgagtcagagccccgccatactgagcgcctcccccggggagaaggtgaccatgacctgtagagccagctccagcctttcatttatgcactggtaccagcagaaacccggtagtagtccaaagccgtggatttacgctacatccaacctggcaagcggagtaccagcccgcttctccggcagcggatcaggaacctcctactccctgacaatcagccgcgtcgaagccgaggatgcagccacatacttttgccaccagtggtcctctaatcccctgacatttggcgcaggcaccaagctcgaactgaagcggggatctaccagcggcagtggaaaacctggtagcggagaggggtctaccaaggggcaagtgcaactcagacagcctggcgcagaactcgtgaagcccggcgcatccgtcaagatgtcttgtaaagccagtggctacaccttcactagctataatatgcactgggttaaacagactcccggtcagggcctcgagtggattggcgcaatctacccgggtaatggtgatacttcttacaatcagaagtttaaggggaaagctaccctgaccgccgacaagtcttcatcaaccgcctacatgcagctgagctctctgacgtctgaggattccgccgtgtattactgcgcccggagccactacgggagtaattatgtcgattattttgactactggggtcagggaacaaccctgactgtctccagctccggaaccacgacgccagcgccgcgaccaccaacaccggcgcccaccatcgcgtcgcagcccctgtccctgcgcccagaggcgtgccggccagcggcggggggcgcagtgcacacgagggggctggacttcgcctgtgatatctacatctgggcgcccttggccgggacttgtggggtccttctcctgtcactggttatcaccctttactgcaaacggggcagaaagaaactcctgtatatattcaaacaaccatttatgagaccagtacaaactactcaagaggaagatggctgtagctgccgatttccagaagaagaagaaggaggatgtgaactgagagtgaagttcagcaggagcgcagacgcccccgcgtacaagcagggccagaaccagctctataacgagctcaatctaggacgaagagaggagtacgatgttttggacaagagacgtggccgggaccctgagatggggggaaagccgagaaggaagaaccctcaggaaggcctgtacaatgaactgcagaaagataagatggcggaggcctacagtgagattgggatgaaaggcgagcgccggaggggcaaggggcacgatggcctttaccagggtctcagtacagccaccaaggacacctacgacgcccttcacatgcaggccctgccccctcgctaag

SEQ ID NO: 18 - DNA, 3680 bp, Artificial Sequence
  pASP30
tcgagttaattaagctagcttacttgtacagctcgtccatgccgagagtgatcccggcggcggtcacgaactccagcaggaccatgtgatcgcgcttctcgttggggtctttgctcagggcggactgggtgctcaggtagtggttgtcgggcagcagcacggggccgtcgccgatgggggtgttctgctggtagtggtcggcgagctgcacgctgccgtcctcgatgttgtggcggatcttgaagttcaccttgatgccgttcttctgcttgtcggccatgatatagacgttgtggctgttgtagttgtactccagcttgtgccccaggatgttgccgtcctccttgaagtcgatgcccttcagctcgatgcggttcaccagggtgtcgccctcgaacttcacctcggcgcgggtcttgtagttgccgtcgtccttgaagaagatggtgcgctcctggacgtagccttcgggcatggcggacttgaagaagtcgtgctgcttcatgtggtcggggtagcggctgaagcactgcacgccgtaggtcagggtggtcacgagggtgggccagggcacgggcagcttgccggtggtgcagatgaacttcagggtcagcttgccgtaggtggcatcgccctcgccctcgccggacacgctgaacttgtggccgtttacgtcgccgtccagctcgaccaggatgggcaccaccccggtgaacagctcctcgcccttgctcaccatggtggctttaccaacagtaccggaatgcccccgggctggaagtcgagcttccattatataccctctaactagtacgccttctgtatgaaacagtttttcctccacgccttctgtatgaaacagtttttcctccacgccttctgtatgaaacagtttttcctccacgccttctgtatgaaacagtttttcctccacgccttctgtatgaaacagtttttcctccacgccttctgtatgaaacagtttttcctccaacagtaccggatgcatcgtgaggctccggtgcccgtcagtgggcagagcgcacatcgcccacagtccccgagaagttggggggaggggtcggcaattgaaccggtgcctagagaaggtggcgcggggtaaactgggaaagtgatgtcgtgtactggctccgcctttttcccgagggtgggggagaaccgtatataagtgcagtagtcgccgtgaacgttctttttcgcaacgggtttgccgccagaacacaggtaagtgccgtgtgtggttcccgcgggcctggcctctttacgggttatggcccttgcgtgccttgaattacttccacctggctgcagtacgtgattcttgatcccgagcttcgggttggaagtgggtgggagagttcgaggccttgcgcttaaggagccccttcgcctcgtgcttgagttgaggcctggcctgggcgctggggccgccgcgtgcgaatctggtggcaccttcgcgcctgtctcgctgctttcgataagtctctagccatttaaaatttttgatgacctgctgcgacgctttttttctggcaagatagtcttgtaaatgcgggccaagatctgcacactggtatttcggtttttggggccgcgggcggcgacggggcccgtgcgtcccagcgcacatgttcggcgaggcggggcctgcgagcgcggccaccgagaatcggacgggggtagtctcaagctggccggcctgctctggtgcctggcctcgcgccgccgtgtatcgccccgccctgggcggcaaggctggcccggtcggcaccagttgcgtgagcggaaagatggccgcttcccggccctgctgcagggagctcaaaatggaggacgcggcgctcgggagagcgggcgggtgagtcacccacacaaaggaaaagggcctttccgtcctcagccgtcgcttcatgtgactccactgagtaccgggcgccgtccaggcacctcgattagttctcgtgcttttggagtacgtcgtctttaggttggggggaggggttttatgcgatggagtttccccacactgagtgggtggagactgaagttaggccagcttggcacttgatgtaattctccttggaatttgccctttttgagtttggatcttggttcattctcaagcctcagacagtggttcaaagtttttttcttccatttcaggtgtcgtgattctagagccaccatggccttaccagtgaccgccttgctcctgccgctggccttgctgctccacgccgccaggccggacattcaaatgacacagagtccctcatccctcagtgccagcgtgggcgatcgggtgactataacctgcagagcttctcaggacgtgaataccgctgtggcgtggtaccagcagaagccaggcaaagcgcctaagcttctcatttatagtgccagcttcctgtactcaggtgttccgtctcgcttttctggaagtagaagtgggaccgatttcacattgacgatcagcagcttgcagcccgaagatttcgccacctactactgtcagcagcactacactaccccaccgacatttggtcaaggcacaaaagtagagattaaacgcactggttccaccagcgggagcgggaaacccggctctggggaggggagcgaggtccagctggtggaatccgggggtggtcttgtgcagccaggaggatccttgaggttgtcctgcgccgcaagcggctttaacatcaaagatacatacatccattgggtccgacaggcccctggaaagggcctggagtgggtcgcccggatctacccaactaacgggtacactcgctacgctgatagcgtcaagggtcggtttactatttctgccgacacctcaaaaaacacagcctacctccagatgaactctctcagagctgaggatacagccgtgtactattgcagccggtggggaggcgacgggttctacgctatggatgtgtgggggcagggcacactggtcaccgtgagctcatccggaaccacgacgccagcgccgcgaccaccaacaccggcgcccaccatcgcgtcgcagcccctgtccctgcgcccagaggcgtgccggccagcggcggggggcgcagtgcacacgagggggctggacttcgcctgtgatatctacatctgggcgcccttggccgggacttgtggggtccttctcctgtcactggttatcaccctttactgcaaacggggcagaaagaaactcctgtatatattcaaacaaccatttatgagaccagtacaaactactcaagaggaagatggctgtagctgccgatttccagaagaagaagaaggaggatgtgaactgagagtgaagttcagcaggagcgcagacgcccccgcgtacaagcagggccagaaccagctctataacgagctcaatctaggacgaagagaggagtacgatgttttggacaagagacgtggccgggaccctgagatggggggaaagccgagaaggaagaaccctcaggaaggcctgtacaatgaactgcagaaagataagatggcggaggcctacagtgagattgggatgaaaggcgagcgccggaggggcaaggggcacgatggcctttaccagggtctcagtacagccaccaaggacacctacgacgcccttcacatgcaggccctgccccctcgctaag

SEQ ID NO: 19 - DNA, 3692 bp, Artificial Sequence
  pASP31
tcgagttaattaagctagcttacttgtacagctcgtccatgccgagagtgatcccggcggcggtcacgaactccagcaggaccatgtgatcgcgcttctcgttggggtctttgctcagggcggactgggtgctcaggtagtggttgtcgggcagcagcacggggccgtcgccgatgggggtgttctgctggtagtggtcggcgagctgcacgctgccgtcctcgatgttgtggcggatcttgaagttcaccttgatgccgttcttctgcttgtcggccatgatatagacgttgtggctgttgtagttgtactccagcttgtgccccaggatgttgccgtcctccttgaagtcgatgcccttcagctcgatgcggttcaccagggtgtcgccctcgaacttcacctcggcgcgggtcttgtagttgccgtcgtccttgaagaagatggtgcgctcctggacgtagccttcgggcatggcggacttgaagaagtcgtgctgcttcatgtggtcggggtagcggctgaagcactgcacgccgtaggtcagggtggtcacgagggtgggccagggcacgggcagcttgccggtggtgcagatgaacttcagggtcagcttgccgtaggtggcatcgccctcgccctcgccggacacgctgaacttgtggccgtttacgtcgccgtccagctcgaccaggatgggcaccaccccggtgaacagctcctcgcccttgctcaccatggtggctttaccaacagtaccggaatgcccccgggctggaagtcgagcttccattatataccctctaactagtacgccttctgtatgaaacagtttttcctccacgccttctgtatgaaacagtttttcctccacgccttctgtatgaaacagtttttcctccacgccttctgtatgaaacagtttttcctccacgccttctgtatgaaacagtttttcctccacgccttctgtatgaaacagtttttcctccaacagtaccggatgcatcgtgaggctccggtgcccgtcagtgggcagagcgcacatcgcccacagtccccgagaagttggggggaggggtcggcaattgaaccggtgcctagagaaggtggcgcggggtaaactgggaaagtgatgtcgtgtactggctccgcctttttcccgagggtgggggagaaccgtatataagtgcagtagtcgccgtgaacgttctttttcgcaacgggtttgccgccagaacacaggtaagtgccgtgtgtggttcccgcgggcctggcctctttacgggttatggcccttgcgtgccttgaattacttccacctggctgcagtacgtgattcttgatcccgagcttcgggttggaagtgggtgggagagttcgaggccttgcgcttaaggagccccttcgcctcgtgcttgagttgaggcctggcctgggcgctggggccgccgcgtgcgaatctggtggcaccttcgcgcctgtctcgctgctttcgataagtctctagccatttaaaatttttgatgacctgctgcgacgctttttttctggcaagatagtcttgtaaatgcgggccaagatctgcacactggtatttcggtttttggggccgcgggcggcgacggggcccgtgcgtcccagcgcacatgttcggcgaggcggggcctgcgagcgcggccaccgagaatcggacgggggtagtctcaagctggccggcctgctctggtgcctggcctcgcgccgccgtgtatcgccccgccctgggcggcaaggctggcccggtcggcaccagttgcgtgagcggaaagatggccgcttcccggccctgctgcagggagctcaaaatggaggacgcggcgctcgggagagcgggcgggtgagtcacccacacaaaggaaaagggcctttccgtcctcagccgtcgcttcatgtgactccactgagtaccgggcgccgtccaggcacctcgattagttctcgtgcttttggagtacgtcgtctttaggttggggggaggggttttatgcgatggagtttccccacactgagtgggtggagactgaagttaggccagcttggcacttgatgtaattctccttggaatttgccctttttgagtttggatcttggttcattctcaagcctcagacagtggttcaaagtttttttcttccatttcaggtgtcgtgattctagagccaccatggccttaccagtgaccgccttgctcctgccgctggccttgctgctccacgccgccaggccggacattcaaatgacacagagtccctcatccctcagtgccagcgtgggcgatcgggtgactataacctgcagagcttctcaggacgtgaataccgctgtggcgtggtaccagcagaagccaggcaaagcgcctaagcttctcatttatagtgccagcttcctgtactcaggtgttccgtctcgcttttctggaagtagaagtgggaccgatttcacattgacgatcagcagcttgcagcccgaagatttcgccacctactactgtcagcagcactacactaccccaccgacatttggtcaaggcacaaaagtagagattaaacgcactggttccaccagcgggagcgggaaacccggctctggggaggggagcgaggtccagctggtggaatccgggggtggtcttgtgcagccaggaggatccttgaggttgtcctgcgccgcaagcggctttaacatcaaagatacatacatccattgggtccgacaggcccctggaaagggcctggagtgggtcgcccggatctacccaactaacgggtacactcgctacgctgatagcgtcaagggtcggtttactatttctgccgacacctcaaaaaacacagcctacctccagatgaactctctcagagctgaggatacagccgtgtactattgcagccggtggggaggcgacgggttctacgctatggatgtgtgggggcagggcacactggtcaccgtgagctcatccggaaccacgacgccagcgccgcgaccaccaacaccggcgcccaccatcgcgtcgcagcccctgtccctgcgcccagaggcgtgccggccagcggcggggggcgcagtgcacacgagggggctggacttcgcctgtgatttttgggtgctggtggtggttggtggagtcctggcttgctatagcttgctagtaacagtggcctttattattttctgggtgaggagtaagaggagcaggctcctgcacagtgactacatgaacatgactccccgccgccccgggcccacccgcaagcattaccagccctatgccccaccacgcgacttcgcagcctatcgctccatcgatagagtgaagttcagcaggagcgcagacgcccccgcgtaccagcagggccagaaccagctctataacgagctcaatctaggacgaagagaggagtacgatgttttggacaagagacgtggccgggaccctgagatggggggaaagccgagaaggaagaaccctcaggaaggcctgtacaatgaactgcagaaagataagatggcggaggcctacagtgagattgggatgaaaggcgagcgccggaggggcaaggggcacgatggcctttaccagggtctcagtacagccaccaaggacacctacgacgcccttcacatgcaggccctgccccctcgctaag

SEQ ID NO: 20 - DNA, 4559 bp, Artificial Sequence
  pASP38
tcgagttaattaagctagcccggtactgttggaggaaaaactgtttcatacagaaggcgtggaggaaaaactgtttcatacagaaggcgtggaggaaaaactgtttcatacagaaggcgtggaggaaaaactgtttcatacagaaggcgtggaggaaaaactgtttcatacagaaggcgtggaggaaaaactgtttcatacagaaggcgtactagttagagggtatataatggaagctcgacttccagcccgggggcattccggtactgttggtaaagccaccatgtgccaccagcagctggtcatcagctggttcagcctggtgttcctggccagccctctggtggccatctgggagctgaagaaagacgtgtacgtggtggaactggactggtatcccgacgcccctggcgagatggtggtgctgacctgcgacacccctgaagaggacggcatcacctggaccctggaccagtctagcgaggtgctgggcagcggcaagaccctgaccatccaggtcaaagagttcggcgacgccggccagtacacctgtcacaagggcggagaggtgctgagccacagcctgctgctgctccacaagaaagaggatggcatttggagcaccgacatcctgaaggaccagaaagagcccaagaacaagaccttcctgagatgcgaggccaagaactacagcggccggttcacctgttggtggctgaccaccatcagcaccgacctgaccttcagcgtgaagtccagcagaggcagcagcgaccctcagggcgtgacatgtggcgccgctacactgtctgccgagagagtgcggggcgacaacaaagagtacgagtacagcgtcgagtgccaggaagatagcgcctgccctgccgccgaggaaagcctgcctatcgaagtgatggtggacgccgtgcacaagctgaagtacgagaactacacctccagctttttcatccgggacatcatcaagcccgaccctcccaagaacctgcagctgaagcctctgaagaacagcagacaggtggaagtgtcctgggagtaccccgacacctggtccacccctcacagctacttcagcctgacattctgtgtgcaagtccagggcaagtccaagcgcgagaaaaaggaccgggtgttcaccgacaagaccagcgccaccgtgatctgccggaagaacgcctctatcagcgtgcgggcccaggaccggtactacagcagctcttggagcgagtgggccagcgtgccatgttctggtggcggaggcggcggaagcagaaatctgccagtggccacccctgaccccggcatgtttccttgtctgcaccacagccagaacctgctgcgggccgtgtccaacatgctgcagaaggcccggcagaccctggaattctacccctgcaccagcgaggaaatcgaccacgaggacatcaccaaggataagaccagcaccgtggaagcctgtctgcccctggaactgaccaagaacgagagctgcctgaacagccgggaaaccagcttcatcaccaacggcagctgtctggccagcagaaagacctccttcatgatggccctgtgcctgagcagcatctacgaggacctgaagatgtaccaggtcgagttcaagaccatgaacgccaagctgctgatggaccccaagcggcagatctttctggaccagaatatgctggccgtgatcgacgagctgatgcaggccctgaacttcaacagcgagacagtgccccagaagtcctccctggaagaacccgacttctacaagaccaagatcaagctgtgcatcctgctgcacgccttccggatcagagccgtgaccatcgacagagtgatgagctacctgaacgcctcctaaatgcatcgtgaggctccggtgcccgtcagtgggcagagcgcacatcgcccacagtccccgagaagttggggggaggggtcggcaattgaaccggtgcctagagaaggtggcgcggggtaaactgggaaagtgatgtcgtgtactggctccgcctttttcccgagggtgggggagaaccgtatataagtgcagtagtcgccgtgaacgttctttttcgcaacgggtttgccgccagaacacaggtaagtgccgtgtgtggttcccgcgggcctggcctctttacgggttatggcccttgcgtgccttgaattacttccacctggctgcagtacgtgattcttgatcccgagcttcgggttggaagtgggtgggagagttcgaggccttgcgcttaaggagccccttcgcctcgtgcttgagttgaggcctggcctgggcgctggggccgccgcgtgcgaatctggtggcaccttcgcgcctgtctcgctgctttcgataagtctctagccatttaaaatttttgatgacctgctgcgacgctttttttctggcaagatagtcttgtaaatgcgggccaagatctgcacactggtatttcggtttttggggccgcgggcggcgacggggcccgtgcgtcccagcgcacatgttcggcgaggcggggcctgcgagcgcggccaccgagaatcggacgggggtagtctcaagctggccggcctgctctggtgcctggcctcgcgccgccgtgtatcgccccgccctgggcggcaaggctggcccggtcggcaccagttgcgtgagcggaaagatggccgcttcccggccctgctgcagggagctcaaaatggaggacgcggcgctcgggagagcgggcgggtgagtcacccacacaaaggaaaagggcctttccgtcctcagccgtcgcttcatgtgactccactgagtaccgggcgccgtccaggcacctcgattagttctcgtgcttttggagtacgtcgtctttaggttggggggaggggttttatgcgatggagtttccccacactgagtgggtggagactgaagttaggccagcttggcacttgatgtaattctccttggaatttgccctttttgagtttggatcttggttcattctcaagcctcagacagtggttcaaagtttttttcttccatttcaggtgtcgtgattctagagccaccatggccttaccagtgaccgccttgctcctgccgctggccttgctgctccacgccgccaggccggacattcaaatgacacagagtccctcatccctcagtgccagcgtgggcgatcgggtgactataacctgcagagcttctcaggacgtgaataccgctgtggcgtggtaccagcagaagccaggcaaagcgcctaagcttctcatttatagtgccagcttcctgtactcaggtgttccgtctcgcttttctggaagtagaagtgggaccgatttcacattgacgatcagcagcttgcagcccgaagatttcgccacctactactgtcagcagcactacactaccccaccgacatttggtcaaggcacaaaagtagagattaaacgcactggttccaccagcgggagcgggaaacccggctctggggaggggagcgaggtccagctggtggaatccgggggtggtcttgtgcagccaggaggatccttgaggttgtcctgcgccgcaagcggctttaacatcaaagatacatacatccattgggtccgacaggcccctggaaagggcctggagtgggtcgcccggatctacccaactaacgggtacactcgctacgctgatagcgtcaagggtcggtttactatttctgccgacacctcaaaaaacacagcctacctccagatgaactctctcagagctgaggatacagccgtgtactattgcagccggtggggaggcgacgggttctacgctatggatgtgtgggggcagggcacactggtcaccgtgagctcatccggaaccacgacgccagcgccgcgaccaccaacaccggcgcccaccatcgcgtcgcagcccctgtccctgcgcccagaggcgtgccggccagcggcggggggcgcagtgcacacgagggggctggacttcgcctgtgatatctacatctgggcgcccttggccgggacttgtggggtccttctcctgtcactggttatcaccctttactgcaaacggggcagaaagaaactcctgtatatattcaaacaaccatttatgagaccagtacaaactactcaagaggaagatggctgtagctgccgatttccagaagaagaagaaggaggatgtgaactgagagtgaagttcagcaggagcgcagacgcccccgcgtacaagcagggccagaaccagctctataacgagctcaatctaggacgaagagaggagtacgatgttttggacaagagacgtggccgggaccctgagatggggggaaagccgagaaggaagaaccctcaggaaggcctgtacaatgaactgcagaaagataagatggcggaggcctacagtgagattgggatgaaaggcgagcgccggaggggcaaggggcacgatggcctttaccagggtctcagtacagccaccaaggacacctacgacgcccttcacatgcaggccctgccccctcgctaag

SEQ ID NO: 21 - DNA, 4505 bp, Artificial Sequence
  pASP52
tcgagttaattaagctagcttacatatgtctcttggcccgcaggtcctcttcggagatcagcttctgctcgcttcccttgccaggagacaggctcagggacttctgggtgtagtggttgtgcagggcctcgtgcatcacgctgcaggagaacacgtttccctgctgccatctgctcttgtccactgtcagcttgctgtacaggaagaatgagccgtcgctgtccagcacaggaggggttgtcttgtagttgttctcaggctggccattgctctcccattccacggcaatgtcgctggggtaaaagcccttgaccaggcaggtcagggacacctgattcttggtcagctcgtccctgcttggaggcagtgtgtaaacctggggttccctaggctggcccttggccttgctgatggttttctcgataggagcaggcagggccttgttggacaccttgcacttgtactctttgccgttcagccaatcctggtgcagcacggtcagcacggacaccactctgtaggtgctgttgtactgttcctctctaggcttggtcttggcgttgtgcacttccacgccgtccacgtaccaattgaacttcacttcggggtcctcgtgagacacatccaccaccacgcaggtcacttcaggggttctgctgatcatcagggtgtccttaggctttggaggaaacaggaacacggaaggtccgccgagcagttctggagcaggacatggaggacaggtgtgggtcttgtcgctgctcttgggttccactttgatttccaccttggtgccctggccaaatgtgtaaggcagggtgttgccctgctggcagtagtaggtggcaatgtcctcaggctgcaggctagatatggtgaaggtgaagtcggtgccgctgccagagccagaaaatctgctgggcacgccgctgtgcagtctgctggtgtagtagatcagcagtttaggggccttgccgggcttttgctgataccaattcaggtagctgctgatgtcctggctggcccgacaggtgattgtcactctgtctcccacagaggcagacaggctgctggggctctgtgtcatctgaatatcgctaccgcctccgccacttcctccgccaccagatcctccgcctccgctagaaacggtgaccagagagccctggccccaataatccatggcggtggttctggccaggcttctggcgcagtagtacacggctgtatcagcagcggtcacgctagacagccgcaggctgaactggttcttgctggtgtctctcagcatggtcactctggacttcaggctgggattgtaggtggtgatgccgctgtagctgatgtagccgatccattccaggcctcttccaggaggttgtcggacccaggaccaggcatgatcgctggtgatgctgtagccggacacggtacaggtcaggctcagtgtttggctaggccgcacgagtccaggtccagactcttgcagctgaacctcgcactgcacgcctctaagcagagccaccaggaacacccagctcaggccgaattccatggtggctttaccaacagtaccggaatgcccccgggctggaagtcgagcttccattatataccctctaactagtacgccttctgtatgaaacagtttttcctccacgccttctgtatgaaacagtttttcctccacgccttctgtatgaaacagtttttcctccacgccttctgtatgaaacagtttttcctccacgccttctgtatgaaacagtttttcctccacgccttctgtatgaaacagtttttcctccaacagtaccggatgcatcgtgaggctccggtgcccgtcagtgggcagagcgcacatcgcccacagtccccgagaagttggggggaggggtcggcaattgaaccggtgcctagagaaggtggcgcggggtaaactgggaaagtgatgtcgtgtactggctccgcctttttcccgagggtgggggagaaccgtatataagtgcagtagtcgccgtgaacgttctttttcgcaacgggtttgccgccagaacacaggtaagtgccgtgtgtggttcccgcgggcctggcctctttacgggttatggcccttgcgtgccttgaattacttccacctggctgcagtacgtgattcttgatcccgagcttcgggttggaagtgggtgggagagttcgaggccttgcgcttaaggagccccttcgcctcgtgcttgagttgaggcctggcctgggcgctggggccgccgcgtgcgaatctggtggcaccttcgcgcctgtctcgctgctttcgataagtctctagccatttaaaatttttgatgacctgctgcgacgctttttttctggcaagatagtcttgtaaatgcgggccaagatctgcacactggtatttcggtttttggggccgcgggcggcgacggggcccgtgcgtcccagcgcacatgttcggcgaggcggggcctgcgagcgcggccaccgagaatcggacgggggtagtctcaagctggccggcctgctctggtgcctggcctcgcgccgccgtgtatcgccccgccctgggcggcaaggctggcccggtcggcaccagttgcgtgagcggaaagatggccgcttcccggccctgctgcagggagctcaaaatggaggacgcggcgctcgggagagcgggcgggtgagtcacccacacaaaggaaaagggcctttccgtcctcagccgtcgcttcatgtgactccactgagtaccgggcgccgtccaggcacctcgattagttctcgtgcttttggagtacgtcgtctttaggttggggggaggggttttatgcgatggagtttccccacactgagtgggtggagactgaagttaggccagcttggcacttgatgtaattctccttggaatttgccctttttgagtttggatcttggttcattctcaagcctcagacagtggttcaaagtttttttcttccatttcaggtgtcgtgattctagaatggccttaccagtgaccgccttgctcctgccgctggccttgctgctccacgccgccaggccgggatccgacatcgttctgagtcagagccccgccatactgagcgcctcccccggggagaaggtgaccatgacctgtagagccagctccagcctttcatttatgcactggtaccagcagaaacccggtagtagtccaaagccgtggatttacgctacatccaacctggcaagcggagtaccagcccgcttctccggcagcggatcaggaacctcctactccctgacaatcagccgcgtcgaagccgaggatgcagccacatacttttgccaccagtggtcctctaatcccctgacatttggcgcaggcaccaagctcgaactgaagcggggatctaccagcggcagtggaaaacctggtagcggagaggggtctaccaaggggcaagtgcaactcagacagcctggcgcagaactcgtgaagcccggcgcatccgtcaagatgtcttgtaaagccagtggctacaccttcactagctataatatgcactgggttaaacagactcccggtcagggcctcgagtggattggcgcaatctacccgggtaatggtgatacttcttacaatcagaagtttaaggggaaagctaccctgaccgccgacaagtcttcatcaaccgcctacatgcagctgagctctctgacgtctgaggattccgccgtgtattactgcgcccggagccactacgggagtaattatgtcgattattttgactactggggtcagggaacaaccctgactgtctccagctccggaaccacgacgccagcgccgcgaccaccaacaccggcgcccaccatcgcgtcgcagcccctgtccctgcgcccagaggcgtgccggccagcggcggggggcgcagtgcacacgagggggctggacttcgcctgtgatatctacatctgggcgcccttggccgggacttgtggggtccttctcctgtcactggttatcaccctttactgcaaacggggcagaaagaaactcctgtatatattcaaacaaccatttatgagaccagtacaaactactcaagaggaagatggctgtagctgccgatttccagaagaagaagaaggaggatgtgaactgagagtgaagttcagcaggagcgcagacgcccccgcgtacaagcagggccagaaccagctctataacgagctcaatctaggacgaagagaggagtacgatgttttggacaagagacgtggccgggaccctgagatggggggaaagccgagaaggaagaaccctcaggaaggcctgtacaatgaactgcagaaagataagatggcggaggcctacagtgagattgggatgaaaggcgagcgccggaggggcaaggggcacgatggcctttaccagggtctcagtacagccaccaaggacacctacgacgcccttcacatgcaggccctgccccctcgctaag

SEQ ID NO: 22 - protein, 509 aa, Artificial Sequence
  anti-hIL-6R scFv-Fc
MEFGLSWVFLVALLRGVQCEVQLQESGPGLVRPSQTLSLTCTVSGYSITSDHAWSWVRQPPGRGLEWIGYISYSGITTYNPSLKSRVTMLRDTSKNQFSLRLSSVTAADTAVYYCARSLARTTAMDYWGQGSLVTVSSGGGGSGGGGSGGGGSDIQMTQSPSSLSASVGDRVTITCRASQDISSYLNWYQQKPGKAPKLLIYYTSRLHSGVPSRFSGSGSGTDFTFTISSLQPEDIATYYCQQGNTLPYTFGQGTKVEIKVEPKSSDKTHTCPPCPAPELLGGPSVFLFPPKPKDTLMISRTPEVTCVVVDVSHEDPEVKFNWYVDGVEVHNAKTKPREEQYNSTYRVVSVLTVLHQDWLNGKEYKCKVSNKALPAPIEKTISKAKGQPREPQVYTLPPSRDELTKNQVSLTCLVKGFYPSDIAVEWESNGQPENNYKTTPPVLDSDGSFFLYSKLTVDKSRWQQGNVFSCSVMHEALHNHYTQKSLSLSPGKGSEQKLISEEDLRAKR

SEQ ID NO: 23 - protein, 495 aa, Artificial Sequence
  Anti-CD20 CAR human
MALPVTALLLPLALLLHAARPGSDIVLSQSPAILSASPGEKVTMTCRASSSLSFMHWYQQKPGSSPKPWIYATSNLASGVPARFSGSGSGTSYSLTISRVEAEDAATYFCHQWSSNPLTFGAGTKLELKRGSTSGSGKPGSGEGSTKGQVQLRQPGAELVKPGASVKMSCKASGYTFTSYNMHWVKQTPGQGLEWIGAIYPGNGDTSYNQKFKGKATLTADKSSSTAYMQLSSLTSEDSAVYYCARSHYGSNYVDYFDYWGQGTTLTVSSSGTTTPAPRPPTPAPTIASQPLSLRPEACRPAAGGAVHTRGLDFACDIYIWAPLAGTCGVLLLSLVITLYCKRGRKKLLYIFKQPFMRPVQTTQEEDGCSCRFPEEEEGGCELRVKFSRSADAPAYKQGQNQLYNELNLGRREEYDVLDKRRGRDPEMGGKPRRKNPQEGLYNELQKDKMAEAYSEIGMKGERRRGKGHDGLYQGLSTATKDTYDALHMQALPPR

SEQ ID NO: 24 - protein, 495 aa, Artificial Sequence
  Anti-CD20 CAR canine
MASRVTALLLPLALLLRAAAASDIVLSQSPAILSASPGEKVTMTCRASSSLSFMHWYQQKPGSSPKPWIYATSNLASGVPARFSGSGSGTSYSLTISRVEAEDAATYFCHQWSSNPLTFGAGTKLELKRGSTSGSGKPGSGEGSTKGQVQLRQPGAELVKPGASVKMSCKASGYTFTSYNMHWVKQTPGQGLEWIGAIYPGNGDTSYNQKFKGKATLTADKSSSTAYMQLSSLTSEDSAVYYCARSHYGSNYVDYFDYWGQGTTLTVSSASPTTPAPRPPTRAPTNASKPVSPRGETCRPAAGSAVKTSGLDFACEIYIWAPLAGTCAVLLLSLVITIICHGRKKLLYLFKQPFMRPVQTAQEEDACSCRFPEEEEGECDLRAKFGRSAAAPEHQQGPNQLYNELNLRGREEYEVLDKRRGLDPEMGGKQRKRNPQEVVYNALQKDKMAEAYSEIGIKSENQRRRGKGHDGLYQGLSTATKDTYDALHMQALPPR

SEQ ID NO: 25 - protein, 490 aa, Artificial Sequence
  Anti-Her2 human CAR with 4-1BB costimulatory domain
MALPVTALLLPLALLLHAARPDIQMTQSPSSLSASVGDRVTITCRASQDVNTAVAWYQQKPGKAPKLLIYSASFLYSGVPSRFSGSRSGTDFTLTISSLQPEDFATYYCQQHYTTPPTFGQGTKVEIKRTGSTSGSGKPGSGEGSEVQLVESGGGLVQPGGSLRLSCAASGFNIKDTYIHWVRQAPGKGLEWVARIYPTNGYTRYADSVKGRFTISADTSKNTAYLQMNSLRAEDTAVYYCSRWGGDGFYAMDVWGQGTLVTVSSSGTTTPAPRPPTPAPTIASQPLSLRPEACRPAAGGAVHTRGLDFACDIYIWAPLAGTCGVLLLSLVITLYCKRGRKKLLYIFKQPFMRPVQTTQEEDGCSCRFPEEEEGGCELRVKFSRSADAPAYKQGQNQLYNELNLGRREEYDVLDKRRGRDPEMGGKPRRKNPQEGLYNELQKDKMAEAYSEIGMKGERRRGKGHDGLYQGLSTATKDTYDALHMQALPPR

SEQ ID NO: 26 - protein, 494 aa, Artificial Sequence
  Anti-Her2 CAR with CD28 costimulatory domain
MALPVTALLLPLALLLHAARPDIQMTQSPSSLSASVGDRVTITCRASQDVNTAVAWYQQKPGKAPKLLIYSASFLYSGVPSRFSGSRSGTDFTLTISSLQPEDFATYYCQQHYTTPPTFGQGTKVEIKRTGSTSGSGKPGSGEGSEVQLVESGGGLVQPGGSLRLSCAASGFNIKDTYIHWVRQAPGKGLEWVARIYPTNGYTRYADSVKGRFTISADTSKNTAYLQMNSLRAEDTAVYYCSRWGGDGFYAMDVWGQGTLVTVSSSGTTTPAPRPPTPAPTIASQPLSLRPEACRPAAGGAVHTRGLDFACDFWVLVVVGGVLACYSLLVTVAFIIFWVRSKRSRLLHSDYMNMTPRRPGPTRKHYQPYAPPRDFAAYRSIDRVKFSRSADAPAYQQGQNQLYNELNLGRREEYDVLDKRRGRDPEMGGKPRRKNPQEGLYNELQKDKMAEAYSEIGMKGERRRGKGHDGLYQGLSTATKDTYDALHMQALPPR

SEQ ID NO: 27 - protein, 532 aa, Artificial Sequence
  hIL-12 (p40-linker-p35)
MCHQQLVISWFSLVFLASPLVAIWELKKDVYVVELDWYPDAPGEMVVLTCDTPEEDGITWTLDQSSEVLGSGKTLTIQVKEFGDAGQYTCHKGGEVLSHSLLLLHKKEDGIWSTDILKDQKEPKNKTFLRCEAKNYSGRFTCWWLTTISTDLTFSVKSSRGSSDPQGVTCGAATLSAERVRGDNKEYEYSVECQEDSACPAAEESLPIEVMVDAVHKLKYENYTSSFFIRDIIKPDPPKNLQLKPLKNSRQVEVSWEYPDTWSTPHSYFSLTFCVQVQGKSKREKKDRVFTDKTSATVICRKNASISVRAQDRYYSSSWSEWASVPCSGGGGGGSRNLPVATPDPGMFPCLHHSQNLLRAVSNMLQKARQTLEFYPCTSEEIDHEDITKDKTSTVEACLPLELTKNESCLNSRETSFITNGSCLASRKTSFMMALCLSSIYEDLKMYQVEFKTMNAKLLMDPKRQIFLDQNMLAVIDELMQALNFNSETVPQKSSLEEPDFYKTKIKLCILLHAFRIRAVTIDRVMSYLNAS

SEQ ID NO: 28 - protein, 533 aa, Artificial Sequence
  cIL-12 (p40-linker-p35)
MHPQQLVISWFSLVLLASSLMTIWELEKDVYVVELDWHPDAPGEMVVLTCHTPEEDDITWTSAQSSEVLGSGKTLTIQVKEFGDAGQYTCHKGGKVLSRSLLLIHKKEDGIWSTDILKEQKESKNKIFLKCEAKNYSGRFTCWWLTAISTDLKFSVKSSRGFSDPQGVTCGAVTLSAERVRVDNRDYKKYTVECQEGSACPSAEESLPIEVVVDAIHKLKYENYTSSFFIRDIIKPDPPTNLQLKPLKNSRHVEVSWEYPDTWSTPHSYFSLTFCVQAQGKNNREKKDRLCVDKTSAKVVCHKDAKIRVQARDRYYSSSWSDWASVSCSGGGGGGSRSLPTASPSPGIFQCLNHSQNLLRAVSNTLQKARQTLELYSCTSEEIDHEDITKDKTSTVEACLPLELTMNESCLASREISLITNGSCLASGKASFMTVLCLSSIYEDLKMYQMEFKAMNAKLLMDPKRQIFLDQNMLTAIDELLQALNFNSVTVPQKSSLEEPDFYKTKIKLCILLHAFRIRAVTIDRMMSYLNSS

SEQ ID NO: 29 - DNA, 23 bp, Artificial Sequence
  Spacer
ggcattccggtactgttggtaaa

SEQ ID NO: 30 - protein, 384 aa, Homo Sapiens
MPQLDSGGGGAGGGDDLGAPDELLAFQDEGEEQDDKSRDSAAGPERDLAELKSSLVNESEGAAGGAGIPGVPGAGAGARGEAEALGREHAAQRLFPDKLPEPLEDGLKAPECTSGMYKETVYSAFNLLMHYPPPSGAGQHPQPQPPLHKANQPPHGVPQLSLYEHFNSPHPTPAPADISQKQVHRPLQTPDLSGFYSLTSGSMGQLPHTVSWFTHPSLMLGSGVPGHPAAIPHPAIVPPSGKQELQPFDRNLKTQAESKAEKEAKKPTIKKPLNAFMLYMKEMRAKVIAECTLKESAAINQILGRRWHALSREEQAKYYELARKERQLHMQLYPGWSARDNYGKKKRRSREKHQESTTETNWPRELKDGNGQESLSMSSSSSPA

SEQ ID NO: 31 - protein, 655 aa, Homo Sapiens
MAEAPQVVEIDPDFEPLPRPRSCAWPLPRPEFSQSNSATSSPAPSGSAAANPDAAAGLPSASAAAVSADFMSNLSLLEESEDFPQAPGSVAAAVAAAAAAAATGGLCGDFQGPEAGCLHPAPPQPPPPGPLSQHPPVPPAAAGPLAGQPRKSSSSRRNAWGNLSYADLITKAIESSAEKRLTLSQIYEWMVKSVPYFKDKGDSNSSAGWKNSIRHNLSLHSKFIRVQNEGTGKSSWWMLNPEGGKSGKSPRRRAAAMDNNSKFAKSRSRAAKKKASLQSGQEGAGDSPGSQFSKWPASPGSHSNDDFDNWSTFRPRTSANASTISGRLSPIMTEQDDLGEGDVHSMVYPPSAAKMASTLPSLSEISNPENMENLLDNLNLLSSPTSLTVSTQSSPGTMMQQTPCYSFAPPNTSLNSPSPNYQKYTYGQSSMSPLPQMPIQTLQDNKSSYGGMSQYNCAPGLLKELLTSDSPPHNDIMTPVDPGVAQPNSRVLGQNVMMGPNSVMSTYGSQASHNKMMNPSSHTHPGHAQQTSAVNGRPLPHTVSTMPHTSGMNRLTQVKTPVQVPLPHPMQMSALGGYSSVSSCNGYGRMGLLHQEKLPSDLDGMFIERLDCDMESIIRNDLMDGDTLDFNFDNVLPNQSFPHSVKTTTHSWVSG

SEQ ID NO: 32 - DNA, 111 bp, Artificial Sequence
  STAT3 responsive element
ccggtactgttagcttcatttcccgtaaatcgtcgaagcttcatttcccgtaaatcgtcgaagcttcatttcccgtaaatcgtcgaagcttcatttcccgtaaatcgtcga

SEQ ID NO: 33 - DNA, 1404 bp, Artificial Sequence
  hIL-6Ra
atgctggccgtgggatgtgctttgcttgctgctctgttggctgctcctggtgctgcactggcccctagaagatgtcctgctcaagaggtggcaagaggcgtgctgacatctctgcctggcgatagcgtgaccctgacatgtcctggcgtggaacccgaggataatgccaccgtgcattgggtgctgagaaagcctgccgccggatctcatcctagcagatgggctggcatgggccgtagactgctgctgagatctgtccagctgcacgacagcggcaactacagctgttacagagccggcagacctgccggaacagtgcatctgctggtggatgtgcctcctgaggaaccccagctgagctgcttcagaaagtcccctctgagcaacgtcgtgtgcgagtggggccctagaagcacacctagcctgacaacaaaggccgtgctgctcgtgcggaagttccagaattctcccgccgaggacttccaagagccttgccagtacagccaagagagccagaagttcagctgtcagctggctgtgcctgagggcgacagcagcttctacatcgtgtctatgtgcgtggccagcagcgtgggcagcaagtttagcaagacccagaccttccaaggctgcggcatcctgcaacctgatcctccagccaacatcaccgtgaccgccgtggccagaaatcccagatggctgtctgtgacctggcaggaccctcacagctggaactccagcttttaccggctgagattcgagctgcggtacagggccgagagaagcaagaccttcaccacctggatggtcaaggacctgcagcatcactgcgtgatccacgatgcttggagcggcctgagacatgtggtgcagctgagagcccaagaggaattcggccaaggcgagtggagtgaatggtcccctgaagccatgggcaccccttggacagagagcagatctccaccagccgagaacgaggtgtccacacctatgcaggccctgaccaccaacaaggacgacgacaacatcctgttccgggacagcgccaatgccacaagtctgcctgtgcaggatagctcctctgtgcccctgcctacctttctggttgctggcggatctctggcctttggcaccctgctgtgtatcgccatcgtgctgcggttcaagaaaacctggaagctgcgggccctgaaagagggcaagacctctatgcaccctccttacagcctgggccagctggtgcctgaaagacctagacctacacctgtgctggtgcccctgatcagccctcctgtgtctccatctagcctgggcagcgacaataccagcagccacaacagacccgacgctcgggaccctagatctccctacgacatcagcaataccgactacttcttcccacgc

SEQ ID NO: 34 - DNA, 1422 bp, Artificial Sequence
  Regulatory unit
aggctggatcggtcccggtgtcttctatggaggtcaaaacagcgtggatggcgtctccaggcgatctgacggttcactaaacgagctctgcttatataggcctcccaccgtacacgcctacggaggacagtactccgtgcggaggacagtactccgtccggaggacagtactccgatcggaggacagtactccggtcggaggacagtactccgctcggaggacagtactccgacgcgtcgtgaggctccggtgcccgtcagtgggcagagcgcacatcgcccacagtccccgagaagttggggggaggggtcggcaattgaaccggtgcctagagaaggtggcgcggggtaaactgggaaagtgatgtcgtgtactggctccgcctttttcccgagggtgggggagaaccgtatataagtgcagtagtcgccgtgaacgttctttttcgcaacgggtttgccgccagaacacaggtaagtgccgtgtgtggttcccgcgggcctggcctctttacgggttatggcccttgcgtgccttgaattacttccacctggctgcagtacgtgattcttgatcccgagcttcgggttggaagtgggtgggagagttcgaggccttgcgcttaaggagccccttcgcctcgtgcttgagttgaggcctggcctgggcgctggggccgccgcgtgcgaatctggtggcaccttcgcgcctgtctcgctgctttcgataagtctctagccatttaaaatttttgatgacctgctgcgacgctttttttctggcaagatagtcttgtaaatgcgggccaagatctgcacactggtatttcggtttttggggccgcgggcggcgacggggcccgtgcgtcccagcgcacatgttcggcgaggcggggcctgcgagcgcggccaccgagaatcggacgggggtagtctcaagctggccggcctgctctggtgcctggcctcgcgccgccgtgtatcgccccgccctgggcggcaaggctggcccggtcggcaccagttgcgtgagcggaaagatggccgcttcccggccctgctgcagggagctcaaaatggaggacgcggcgctcgggagagcgggcgggtgagtcacccacacaaaggaaaagggcctttccgtcctcagccgtcgcttcatgtgactccactgagtaccgggcgccgtccaggcacctcgattagttctcgtgcttttggagtacgtcgtctttaggttggggggaggggttttatgcgatggagtttccccacactgagtgggtggagactgaagttaggccagcttggcacttgatgtaattctccttggaatttgccctttttgagtttggatcttggttcattctcaagcctcagacagtggttcaaagtttttttcttccatttcaggtgtcgtga

SEQ ID NO: 35 - protein, 236 aa, Artificial Sequence
  mCherry reporter
MVSKGEEDNMAIIKEFMRFKVHMEGSVNGHEFEIEGEGEGRPYEGTQTAKLKVTKGGPLPFAWDILSPQFMYGSKAYVKHPADIPDYLKLSFPEGFKWERVMNFEDGGVVTVTQDSSLQDGEFIYKVKLRGTNFPSDGPVMQKKTMGWEASSERMYPEDGALKGEIKQRLKLKDGGHYDAEVKTTYKAKKPVQLPGAYNVNIKLDITSHNEDYTIVEQYERAEGRHSTGGMDELYK

SEQ ID NO: 36 - protein, 781 aa, Artificial Sequence
  4D5-Notch1-Gal4-VP64 receptor
DIQMTQSPSSLSASVGDRVTITCRASQDVNTAVAWYQQKPGKAPKLLIYSASFLYSGVPSRFSGSRSGTDFTLTISSLQPEDFATYYCQQHYTTPPTFGQGTKVEIKRTGSTSGSGKPGSGEGSEVQLVESGGGLVQPGGSLRLSCAASGFNIKDTYIHWVRQAPGKGLEWVARIYPTNGYTRYADSVKGRFTISADTSKNTAYLQMNSLRAEDTAVYYCSRWGGDGFYAMDVWGQGTLVTVSSILDYSFTGGAGRDIPPPQIEEACELPECQVDAGNKVCNLQCNNHACGWDGGDCSLNFNDPWKNCTQSLQCWKYFSDGHCDSQCNSAGCLFDGFDCQLTEGQCNPLYDQYCKDHFSDGHCDQGCNSAECEWDGLDCAEHVPERLAAGTLVLVVLLPPDQLRNNSFHFLRELSHVLHTNVVFKRDAQGQQMIFPYYGHEEELRKHPIKRSTVGWATSSLLPGTSGGRQRRELDPMDIRGSIVYLEIDNRQCVQSSSQCFQSATDVAAFLGALASLGSLNIPYKIEAVKSEPVEPPLPSQLHLMYVAAAAFVLLFFVGCGVLLSRKRRRMKLLSSIEQACDICRLKKLKCSKEKPKCAKCLKNNWECRYSPKTKRSPLTRAHLTEVESRLERLEQLFLLIFPREDLDMILKMDSLQDIKALLTGLFVQDNVNKDAVTDRLASVETDMPLTLRQHRISATSSSEESSNKGQRQLTVSAAAGGSGGSGGSDALDDFDLDMLGSDALDDFDLDMLGSDALDDFDLDMLGSDALDDFDLDMLGS

SEQ ID NO: 37 - protein, 233 aa, Artificial Sequence
  BFP2 reporter
MSELIKENMHMKLYMEGTVDNHHFKCTSEGEGKPYEGTQTMRIKVVEGGPLPFAFDILATSFLYGSKTFINHTQGIPDFFKQSFPEGFTWERVTTYEDGGVLTATQDTSLQDGCLIYNVKIRGVNFTSNGPVMQKKTLGWEAFTETLYPADGGLEGRNDMALKLVGGSHLIANAKTTYRSKKPAKNLKMPGVYYVDYRLERIKEANNETYVEQHEVAVARYCDLPSKLGHKLN

SEQ ID NO: 38 - protein, 655 aa, Homo Sapiens
MAEAPQVVEIDPDFEPLPRPRSCTWPLPRPEFSQSNSATSSPAPSGSAAANPDAAAGLPSASAAAVSADFMSNLSLLEESEDFPQAPGSVAAAVAAAAAAAATGGLCGDFQGPEAGCLHPAPPQPPPPGPLSQHPPVPPAAAGPLAGQPRKSSSSRRNAWGNLSYADLITKAIESSAEKRLTLSQIYEWMVKSVPYFKDKGDSNSSAGWKNSIRHNLSLHSKFIRVQNEGTGKSSWWMLNPEGGKSGKSPRRRAASMDNNSKFAKSRSRAAKKKASLQSGQEGAGDSPGSQFSKWPASPGSHSNDDFDNWSTFRPRTSSNASTISGRLSPIMTEQDDLGEGDVHSMVYPPSAAKMASTLPSLSEISNPENMENLLDNLNLLSSPTSLTVSTQSSPGTMMQQTPCYSFAPPNTSLNSPSPNYQKYTYGQSSMSPLPQMPIQTLQDNKSSYGGMSQYNCAPGLLKELLTSDSPPHNDIMTPVDPGVAQPNSRVLGQNVMMGPNSVMSTYGSQASHNKMMNPSSHTHPGHAQQTSAVNGRPLPHTVSTMPHTSGMNRLTQVKTPVQVPLPHPMQMSALGGYSSVSSCNGYGRMGLLHQEKLPSDLDGMFIERLDCDMESIIRNDLMDGDTLDFNFDNVLPNQSFPHSVKTTTHSWVSG

SEQ ID NO: 39 - DNA, 20 bp, Artificial Sequence
  TRAC
tgtgctagacatgaggtcta

SEQ ID NO: 40 - DNA, 20 bp, Artificial Sequence
  TRBC
ggagaatgacgagtggaccc